European Patent Application EP 4 242 308 A1, published September 13, 2023. Title: SARS-CoV-2 mRNA Vaccine and Preparation Method and Use Thereof. Applicant: Shenzhen Rhegen Biotechnology Co., Ltd. The sequence listing filed with the application follows.

SEQUENCE LISTING (55 sequences)

SEQ ID NO: 1 - protein, 541 aa, synthetic construct
  REGION 1..541: note = Antigen
MFVFLVLLPLVSSQCVNLTTRTQLPPAYTNSFTRGVYYPDKVFRSSVLHSTQDLFLPFFSNVTWFHAIHVSGTNGTKRFDNPVLPFNDGVYFASTEKSNIIRGWIFGTTLDSKTQSLLIVNNATNVVIKVCEFQFCNDPFLGVYYHKNNKSWMESEFRVYSSANNCTFEYVSQPFLMDLEGKQGNFKNLREFVFKNIDGYFKIYSKHTPINLVRDLPQGFSALEPLVDLPIGINITRFQTLLALHRSYLTPGDSSSGWTAGAAAYYVGYLQPRTFLLKYNENGTITDAVDCALDPLSETKCTLKSFTVEKGIYQTSNFRVQPTESIVRFPNITNLCPFGEVFNATRFASVYAWNRKRISNCVADYSVLYNSASFSTFKCYGVSPTKLNDLCFTNVYADSFVIRGDEVRQIAPGQTGKIADYNYKLPDDFTGCVIAWNSNNLDSKVGGNYNYLYRLFRKSNLKPFERDISTEIYQAGSTPCNGVEGFNCYFPLQSYGFQPTNGVGYQPYRVVVLSFELLHAPATVCGPKKSTNLVKNKCVNF

SEQ ID NO: 2 - DNA, 1623 bp, synthetic construct
  misc_feature 1..1623: note = For the preparation of mRNA vaccines
  source 1..1623: mol_type = other DNA
atgttcgtgttcctggtgctgctgcccctggtgagcagccagtgcgtgaacctgaccaccaggacccagctgccccccgcctacaccaacagcttcaccaggggcgtgtactaccccgacaaggtgttcaggagcagcgtgctgcacagcacccaggacctgttcctgcccttcttcagcaacgtgacctggttccacgccatccacgtgagcggcaccaacggcaccaagaggttcgacaaccccgtgctgcccttcaacgacggcgtgtacttcgccagcaccgagaagagcaacatcatcaggggctggatcttcggcaccaccctggacagcaagacccagagcctgctgatcgtgaacaacgccaccaacgtggtgatcaaggtgtgcgagttccagttctgcaacgaccccttcctgggcgtgtactaccacaagaacaacaagagctggatggagagcgagttcagggtgtacagcagcgccaacaactgcaccttcgagtacgtgagccagcccttcctgatggacctggagggcaagcagggcaacttcaagaacctgagggagttcgtgttcaagaacatcgacggctacttcaagatctacagcaagcacacccccatcaacctggtgagggacctgccccagggcttcagcgccctggagcccctggtggacctgcccatcggcatcaacatcaccaggttccagaccctgctggccctgcacaggagctacctgacccccggcgacagcagcagcggctggaccgccggcgccgccgcctactacgtgggctacctgcagcccaggaccttcctgctgaagtacaacgagaacggcaccatcaccgacgccgtggactgcgccctggaccccctgagcgagaccaagtgcaccctgaagagcttcaccgtggagaagggcatctaccagaccagcaacttcagggtgcagcccaccgagagcatcgtgaggttccccaacatcaccaacctgtgccccttcggcgaggtgttcaacgccaccaggttcgccagcgtgtacgcctggaacaggaagaggatcagcaactgcgtggccgactacagcgtgctgtacaacagcgccagcttcagcaccttcaagtgctacggcgtgagccccaccaagctgaacgacctgtgcttcaccaacgtgtacgccgacagcttcgtgatcaggggcgacgaggtgaggcagatcgcccccggccagaccggcaagatcgccgactacaactacaagctgcccgacgacttcaccggctgcgtgatcgcctggaacagcaacaacctggacagcaaggtgggcggcaactacaactacctgtacaggctgttcaggaagagcaacctgaagcccttcgagagggacatcagcaccgagatctaccaggccggcagcaccccctgcaacggcgtggagggcttcaactgctacttccccctgcagagctacggcttccagcccaccaacggcgtgggctaccagccctacagggtggtggtgctgagcttcgagctgctgcacgcccccgccaccgtgtgcggccccaagaagagcaccaacctggtgaagaacaagtgcgtgaacttc

SEQ ID NO: 3 - DNA, 1623 bp, synthetic construct
  misc_feature 1..1623: note = For the preparation of mRNA vaccines
  source 1..1623: mol_type = other DNA
atgttcgtgttcctggtgctgctgcctctggtgagcagccagtgcgtgaacctgaccaccagaacccagctgcctcctgcctacaccaacagcttcaccagaggcgtgtactaccctgacaaggtgttcagaagcagcgtgctgcacagcacccaggacctgttcctgcctttcttcagcaacgtgacctggttccacgccatccacgtgagcggcaccaacggcaccaagagattcgacaaccctgtgctgcctttcaacgacggcgtgtacttcgccagcaccgagaagagcaacatcatcagaggctggatcttcggcaccaccctggacagcaagacccagagcctgctgatcgtgaacaacgccaccaacgtggtgatcaaggtgtgcgagttccagttctgcaacgaccctttcctgggcgtgtactaccacaagaacaacaagagctggatggagagcgagttcagagtgtacagcagcgccaacaactgcaccttcgagtacgtgagccagcctttcctgatggacctggagggcaagcagggcaacttcaagaacctgagagagttcgtgttcaagaacatcgacggctacttcaagatctacagcaagcacacccctatcaacctggtgagagacctgcctcagggcttcagcgccctggagcctctggtggacctgcctatcggcatcaacatcaccagattccagaccctgctggccctgcacagaagctacctgacccctggcgacagcagcagcggctggaccgccggcgccgccgcctactacgtgggctacctgcagcctagaaccttcctgctgaagtacaacgagaacggcaccatcaccgacgccgtggactgcgccctggaccctctgagcgagaccaagtgcaccctgaagagcttcaccgtggagaagggcatctaccagaccagcaacttcagagtgcagcctaccgagagcatcgtgagattccctaacatcaccaacctgtgccctttcggcgaggtgttcaacgccaccagattcgccagcgtgtacgcctggaacagaaagagaatcagcaactgcgtggccgactacagcgtgctgtacaacagcgccagcttcagcaccttcaagtgctacggcgtgagccctaccaagctgaacgacctgtgcttcaccaacgtgtacgccgacagcttcgtgatcagaggcgacgaggtgagacagatcgcccctggccagaccggcaagatcgccgactacaactacaagctgcctgacgacttcaccggctgcgtgatcgcctggaacagcaacaacctggacagcaaggtgggcggcaactacaactacctgtacagactgttcagaaagagcaacctgaagcctttcgagagagacatcagcaccgagatctaccaggccggcagcaccccttgcaacggcgtggagggcttcaactgctacttccctctgcagagctacggcttccagcctaccaacggcgtgggctaccagccttacagagtggtggtgctgagcttcgagctgctgcacgcccctgccaccgtgtgcggccctaagaagagcaccaacctggtgaagaacaagtgcgtgaacttc

SEQ ID NO: 4 - DNA, 1623 bp, synthetic construct; identical to SEQ ID NO: 2
  misc_feature 1..1623: note = For the preparation of mRNA vaccines
  source 1..1623: mol_type = other DNA

SEQ ID NO: 5 - protein, 538 aa, synthetic construct
  REGION 1..538: note = Antigen
MFVFLVLLPLVSSQCVNLTTRTQLPPAYTNSFTRGVYYPDKVFRSSVLHSTQDLFLPFFSNVTWFHAISGTNGTKRFDNPVLPFNDGVYFASTEKSNIIRGWIFGTTLDSKTQSLLIVNNATNVVIKVCEFQFCNDPFLGVYHKNNKSWMESEFRVYSSANNCTFEYVSQPFLMDLEGKQGNFKNLREFVFKNIDGYFKIYSKHTPINLVRDLPQGFSALEPLVDLPIGINITRFQTLLALHRSYLTPGDSSSGWTAGAAAYYVGYLQPRTFLLKYNENGTITDAVDCALDPLSETKCTLKSFTVEKGIYQTSNFRVQPTESIVRFPNITNLCPFGEVFNATRFASVYAWNRKRISNCVADYSVLYNSASFSTFKCYGVSPTKLNDLCFTNVYADSFVIRGDEVRQIAPGQTGKIADYNYKLPDDFTGCVIAWNSNNLDSKVGGNYNYLYRLFRKSNLKPFERDISTEIYQAGSTPCNGVEGFNCYFPLQSYGFQPTYGVGYQPYRVVVLSFELLHAPATVCGPKKSTNLVKNKCVNF

SEQ ID NO: 6 - DNA, 1614 bp, synthetic construct
  misc_feature 1..1614: note = For the preparation of mRNA vaccines
  source 1..1614: mol_type = other DNA
atgttcgtgttcctggtgctgctgcccctggtgagcagccagtgcgtgaacctgaccaccagaacccagctgccccccgcctacaccaacagcttcaccagaggcgtgtactaccccgacaaggtgttcagaagcagcgtgctgcacagcacccaggacctgttcctgcccttcttcagcaacgtgacctggttccacgccatcagcggcaccaacggcaccaagagattcgacaaccccgtgctgcccttcaacgacggcgtgtacttcgccagcaccgagaagagcaacatcatcagaggctggatcttcggcaccaccctggacagcaagacccagagcctgctgatcgtgaacaacgccaccaacgtggtgatcaaggtgtgcgagttccagttctgcaacgaccccttcctgggcgtgtaccacaagaacaacaagagctggatggagagcgagttcagagtgtacagcagcgccaacaactgcaccttcgagtacgtgagccagcccttcctgatggacctggagggcaagcagggcaacttcaagaacctgagagagttcgtgttcaagaacatcgacggctacttcaagatctacagcaagcacacccccatcaacctggtgagagacctgccccagggcttcagcgccctggagcccctggtggacctgcccatcggcatcaacatcaccagattccagaccctgctggccctgcacagaagctacctgacccccggcgacagcagcagcggctggaccgccggcgccgccgcctactacgtgggctacctgcagcccagaaccttcctgctgaagtacaacgagaacggcaccatcaccgacgccgtggactgcgccctggaccccctgagcgagaccaagtgcaccctgaagagcttcaccgtggagaagggcatctaccagaccagcaacttcagagtgcagcccaccgagagcatcgtgagattccccaacatcaccaacctgtgccccttcggcgaggtgttcaacgccaccagattcgccagcgtgtacgcctggaacagaaagagaatcagcaactgcgtggccgactacagcgtgctgtacaacagcgccagcttcagcaccttcaagtgctacggcgtgagccccaccaagctgaacgacctgtgcttcaccaacgtgtacgccgacagcttcgtgatcagaggcgacgaggtgagacagatcgcccccggccagaccggcaagatcgccgactacaactacaagctgcccgacgacttcaccggctgcgtgatcgcctggaacagcaacaacctggacagcaaggtgggcggcaactacaactacctgtacagactgttcagaaagagcaacctgaagcccttcgagagagacatcagcaccgagatctaccaggccggcagcaccccctgcaacggcgtggagggcttcaactgctacttccccctgcagagctacggcttccagcccacctacggcgtgggctaccagccctacagagtggtggtgctgagcttcgagctgctgcacgcccccgccaccgtgtgcggccccaagaagagcaccaacctggtgaagaacaagtgcgtgaacttc

SEQ ID NO: 7 - DNA, 1614 bp, synthetic construct
  misc_feature 1..1614: note = For the preparation of mRNA vaccines
  source 1..1614: mol_type = other DNA
atgttcgtgttcctggtgctgctgcctctggtgagcagccagtgcgtgaacctgaccaccagaacccagctgcctcctgcctacaccaacagcttcaccagaggcgtgtactaccctgacaaggtgttcagaagcagcgtgctgcacagcacccaggacctgttcctgcctttcttcagcaacgtgacctggttccacgccatcagcggcaccaacggcaccaagagattcgacaaccctgtgctgcctttcaacgacggcgtgtacttcgccagcaccgagaagagcaacatcatcagaggctggatcttcggcaccaccctggacagcaagacccagagcctgctgatcgtgaacaacgccaccaacgtggtgatcaaggtgtgcgagttccagttctgcaacgaccctttcctgggcgtgtaccacaagaacaacaagagctggatggagagcgagttcagagtgtacagcagcgccaacaactgcaccttcgagtacgtgagccagcctttcctgatggacctggagggcaagcagggcaacttcaagaacctgagagagttcgtgttcaagaacatcgacggctacttcaagatctacagcaagcacacccctatcaacctggtgagagacctgcctcagggcttcagcgccctggagcctctggtggacctgcctatcggcatcaacatcaccagattccagaccctgctggccctgcacagaagctacctgacccctggcgacagcagcagcggctggaccgccggcgccgccgcctactacgtgggctacctgcagcctagaaccttcctgctgaagtacaacgagaacggcaccatcaccgacgccgtggactgcgccctggaccctctgagcgagaccaagtgcaccctgaagagcttcaccgtggagaagggcatctaccagaccagcaacttcagagtgcagcctaccgagagcatcgtgagattccctaacatcaccaacctgtgccctttcggcgaggtgttcaacgccaccagattcgccagcgtgtacgcctggaacagaaagagaatcagcaactgcgtggccgactacagcgtgctgtacaacagcgccagcttcagcaccttcaagtgctacggcgtgagccctaccaagctgaacgacctgtgcttcaccaacgtgtacgccgacagcttcgtgatcagaggcgacgaggtgagacagatcgcccctggccagaccggcaagatcgccgactacaactacaagctgcctgacgacttcaccggctgcgtgatcgcctggaacagcaacaacctggacagcaaggtgggcggcaactacaactacctgtacagactgttcagaaagagcaacctgaagcctttcgagagagacatcagcaccgagatctaccaggccggcagcaccccttgcaacggcgtggagggcttcaactgctacttccctctgcagagctacggcttccagcctacctacggcgtgggctaccagccttacagagtggtggtgctgagcttcgagctgctgcacgcccctgccaccgtgtgcggccctaagaagagcaccaacctggtgaagaacaagtgcgtgaacttc

SEQ ID NO: 8 - DNA, 1614 bp, synthetic construct
  misc_feature 1..1614: note = For the preparation of mRNA vaccines
  source 1..1614: mol_type = other DNA
atgttcgtgttcctggtgctgctgcccctggtgagcagccagtgcgtgaacctgaccaccaggacccagctgccccccgcctacaccaacagcttcaccaggggcgtgtactaccccgacaaggtgttcaggagcagcgtgctgcacagcacccaggacctgttcctgcccttcttcagcaacgtgacctggttccacgccatcagcggcaccaacggcaccaagaggttcgacaaccccgtgctgcccttcaacgacggcgtgtacttcgccagcaccgagaagagcaacatcatcaggggctggatcttcggcaccaccctggacagcaagacccagagcctgctgatcgtgaacaacgccaccaacgtggtgatcaaggtgtgcgagttccagttctgcaacgaccccttcctgggcgtgtaccacaagaacaacaagagctggatggagagcgagttcagggtgtacagcagcgccaacaactgcaccttcgagtacgtgagccagcccttcctgatggacctggagggcaagcagggcaacttcaagaacctgagggagttcgtgttcaagaacatcgacggctacttcaagatctacagcaagcacacccccatcaacctggtgagggacctgccccagggcttcagcgccctggagcccctggtggacctgcccatcggcatcaacatcaccaggttccagaccctgctggccctgcacaggagctacctgacccccggcgacagcagcagcggctggaccgccggcgccgccgcctactacgtgggctacctgcagcccaggaccttcctgctgaagtacaacgagaacggcaccatcaccgacgccgtggactgcgccctggaccccctgagcgagaccaagtgcaccctgaagagcttcaccgtggagaagggcatctaccagaccagcaacttcagggtgcagcccaccgagagcatcgtgaggttccccaacatcaccaacctgtgccccttcggcgaggtgttcaacgccaccaggttcgccagcgtgtacgcctggaacaggaagaggatcagcaactgcgtggccgactacagcgtgctgtacaacagcgccagcttcagcaccttcaagtgctacggcgtgagccccaccaagctgaacgacctgtgcttcaccaacgtgtacgccgacagcttcgtgatcaggggcgacgaggtgaggcagatcgcccccggccagaccggcaagatcgccgactacaactacaagctgcccgacgacttcaccggctgcgtgatcgcctggaacagcaacaacctggacagcaaggtgggcggcaactacaactacctgtacaggctgttcaggaagagcaacctgaagcccttcgagagggacatcagcaccgagatctaccaggccggcagcaccccctgcaacggcgtggagggcttcaactgctacttccccctgcagagctacggcttccagcccacctacggcgtgggctaccagccctacagggtggtggtgctgagcttcgagctgctgcacgcccccgccaccgtgtgcggccccaagaagagcaccaacctggtgaagaacaagtgcgtgaacttc

SEQ ID NO: 9 - protein, 539 aa, synthetic construct
  REGION 1..539: note = Antigen
MFVFLVLLPLVSSQCVNLTTRTQLPPAYTNSFTRGVYYPDKVFRSSVLHSTQDLFLPFFSNVTWFHAIHVSGTNGTKRFANPVLPFNDGVYFASTEKSNIIRGWIFGTTLDSKTQSLLIVNNATNVVIKVCEFQFCNDPFLGVYYHKNNKSWMESEFRVYSSANNCTFEYVSQPFLMDLEGKQGNFKNLREFVFKNIDGYFKIYSKHTPINLVRGLPQGFSALEPLVDLPIGINITRFQTLLHRSYLTPGDSSSGWTAGAAAYYVGYLQPRTFLLKYNENGTITDAVDCALDPLSETKCTLKSFTVEKGIYQTSNFRVQPTESIVRFPNITNLCPFGEVFNATRFASVYAWNRKRISNCVADYSVLYNSASFSTFKCYGVSPTKLNDLCFTNVYADSFVIRGDEVRQIAPGQTGNIADYNYKLPDDFTGCVIAWNSNNLDSKVGGNYNYLYRLFRKSNLKPFERDISTEIYQAGSTPCNGVKGFNCYFPLQSYGFQPTYGVGYQPYRVVVLSFELLHAPATVCGPKKSTNLVKNKCVNF

SEQ ID NO: 10 - DNA, 1617 bp, synthetic construct
  misc_feature 1..1617: note = For the preparation of mRNA vaccines
  source 1..1617: mol_type = other DNA
atgttcgtgttcctggtgctgctgcccctggtgagcagccagtgcgtgaacctgaccaccaggacccagctgccccccgcctacaccaacagcttcaccaggggcgtgtactaccccgacaaggtgttcaggagcagcgtgctgcacagcacccaggacctgttcctgcccttcttcagcaacgtgacctggttccacgccatccacgtgagcggcaccaacggcaccaagaggttcgccaaccccgtgctgcccttcaacgacggcgtgtacttcgccagcaccgagaagagcaacatcatcaggggctggatcttcggcaccaccctggacagcaagacccagagcctgctgatcgtgaacaacgccaccaacgtggtgatcaaggtgtgcgagttccagttctgcaacgaccccttcctgggcgtgtactaccacaagaacaacaagagctggatggagagcgagttcagggtgtacagcagcgccaacaactgcaccttcgagtacgtgagccagcccttcctgatggacctggagggcaagcagggcaacttcaagaacctgagggagttcgtgttcaagaacatcgacggctacttcaagatctacagcaagcacacccccatcaacctggtgaggggcctgccccagggcttcagcgccctggagcccctggtggacctgcccatcggcatcaacatcaccaggttccagaccctgctgcacaggagctacctgacccccggcgacagcagcagcggctggaccgccggcgccgccgcctactacgtgggctacctgcagcccaggaccttcctgctgaagtacaacgagaacggcaccatcaccgacgccgtggactgcgccctggaccccctgagcgagaccaagtgcaccctgaagagcttcaccgtggagaagggcatctaccagaccagcaacttcagggtgcagcccaccgagagcatcgtgaggttccccaacatcaccaacctgtgccccttcggcgaggtgttcaacgccaccaggttcgccagcgtgtacgcctggaacaggaagaggatcagcaactgcgtggccgactacagcgtgctgtacaacagcgccagcttcagcaccttcaagtgctacggcgtgagccccaccaagctgaacgacctgtgcttcaccaacgtgtacgccgacagcttcgtgatcaggggcgacgaggtgaggcagatcgcccccggccagaccggcaacatcgccgactacaactacaagctgcccgacgacttcaccggctgcgtgatcgcctggaacagcaacaacctggacagcaaggtgggcggcaactacaactacctgtacaggctgttcaggaagagcaacctgaagcccttcgagagggacatcagcaccgagatctaccaggccggcagcaccccctgcaacggcgtgaagggcttcaactgctacttccccctgcagagctacggcttccagcccacctacggcgtgggctaccagccctacagggtggtggtgctgagcttcgagctgctgcacgcccccgccaccgtgtgcggccccaagaagagcaccaacctggtgaagaacaagtgcgtgaacttc

SEQ ID NO: 11 - DNA, 1617 bp, synthetic construct
  misc_feature 1..1617: note = For the preparation of mRNA vaccines
  source 1..1617: mol_type = other DNA
atgttcgtgttcctggtgctgctgcctctggtgagcagccagtgcgtgaacctgaccaccaggacccagctgcctcctgcctacaccaacagcttcaccaggggcgtgtactaccctgacaaggtgttcaggagcagcgtgctgcacagcacccaggacctgttcctgcctttcttcagcaacgtgacctggttccacgccatccacgtgagcggcaccaacggcaccaagaggttcgccaaccctgtgctgcctttcaacgacggcgtgtacttcgccagcaccgagaagagcaacatcatcaggggctggatcttcggcaccaccctggacagcaagacccagagcctgctgatcgtgaacaacgccaccaacgtggtgatcaaggtgtgcgagttccagttctgcaacgaccctttcctgggcgtgtactaccacaagaacaacaagagctggatggagagcgagttcagggtgtacagcagcgccaacaactgcaccttcgagtacgtgagccagcctttcctgatggacctggagggcaagcagggcaacttcaagaacctgagggagttcgtgttcaagaacatcgacggctacttcaagatctacagcaagcacacccctatcaacctggtgaggggcctgcctcagggcttcagcgccctggagcctctggtggacctgcctatcggcatcaacatcaccaggttccagaccctgctgcacaggagctacctgacccctggcgacagcagcagcggctggaccgccggcgccgccgcctactacgtgggctacctgcagcctaggaccttcctgctgaagtacaacgagaacggcaccatcaccgacgccgtggactgcgccctggaccctctgagcgagaccaagtgcaccctgaagagcttcaccgtggagaagggcatctaccagaccagcaacttcagggtgcagcctaccgagagcatcgtgaggttccctaacatcaccaacctgtgccctttcggcgaggtgttcaacgccaccaggttcgccagcgtgtacgcctggaacaggaagaggatcagcaactgcgtggccgactacagcgtgctgtacaacagcgccagcttcagcaccttcaagtgctacggcgtgagccctaccaagctgaacgacctgtgcttcaccaacgtgtacgccgacagcttcgtgatcaggggcgacgaggtgaggcagatcgcccctggccagaccggcaacatcgccgactacaactacaagctgcctgacgacttcaccggctgcgtgatcgcctggaacagcaacaacctggacagcaaggtgggcggcaactacaactacctgtacaggctgttcaggaagagcaacctgaagcctttcgagagggacatcagcaccgagatctaccaggccggcagcaccccttgcaacggcgtgaagggcttcaactgctacttccctctgcagagctacggcttccagcctacctacggcgtgggctaccagccttacagggtggtggtgctgagcttcgagctgctgcacgcccctgccaccgtgtgcggccctaagaagagcaccaacctggtgaagaacaagtgcgtgaacttc

SEQ ID NO: 12 - DNA, 1617 bp, synthetic construct; identical to SEQ ID NO: 10
  misc_feature 1..1617: note = For the preparation of mRNA vaccines
  source 1..1617: mol_type = other DNA

SEQ ID NO: 13 - protein, 541 aa, synthetic construct
  REGION 1..541: note = Antigen
MFVFLVLLPLVSSQCVNFTNRTQLPSAYTNSFTRGVYYPDKVFRSSVLHSTQDLFLPFFSNVTWFHAIHVSGTNGTKRFDNPVLPFNDGVYFASTEKSNIIRGWIFGTTLDSKTQSLLIVNNATNVVIKVCEFQFCNYPFLGVYYHKNNKSWMESEFRVYSSANNCTFEYVSQPFLMDLEGKQGNFKNLSEFVFKNIDGYFKIYSKHTPINLVRDLPQGFSALEPLVDLPIGINITRFQTLLALHRSYLTPGDSSSGWTAGAAAYYVGYLQPRTFLLKYNENGTITDAVDCALDPLSETKCTLKSFTVEKGIYQTSNFRVQPTESIVRFPNITNLCPFGEVFNATRFASVYAWNRKRISNCVADYSVLYNSASFSTFKCYGVSPTKLNDLCFTNVYADSFVIRGDEVRQIAPGQTGTIADYNYKLPDDFTGCVIAWNSNNLDSKVGGNYNYLYRLFRKSNLKPFERDISTEIYQAGSTPCNGVKGFNCYFPLQSYGFQPTYGVGYQPYRVVVLSFELLHAPATVCGPKKSTNLVKNKCVNF

SEQ ID NO: 14 - DNA, 1623 bp, synthetic construct
  misc_feature 1..1623: note = For the preparation of mRNA vaccines
  source 1..1623: mol_type = other DNA
atgttcgtgttcctggtgctgctgcccctggtgagcagccagtgcgtgaacttcaccaacagaacccagctgcccagcgcctacaccaacagcttcaccagaggcgtgtactaccccgacaaggtgttcagaagcagcgtgctgcacagcacccaggacctgttcctgcccttcttcagcaacgtgacctggttccacgccatccacgtgagcggcaccaacggcaccaagagattcgacaaccccgtgctgcccttcaacgacggcgtgtacttcgccagcaccgagaagagcaacatcatcagaggctggatcttcggcaccaccctggacagcaagacccagagcctgctgatcgtgaacaacgccaccaacgtggtgatcaaggtgtgcgagttccagttctgcaactaccccttcctgggcgtgtactaccacaagaacaacaagagctggatggagagcgagttcagagtgtacagcagcgccaacaactgcaccttcgagtacgtgagccagcccttcctgatggacctggagggcaagcagggcaacttcaagaacctgagcgagttcgtgttcaagaacatcgacggctacttcaagatctacagcaagcacacccccatcaacctggtgagagacctgccccagggcttcagcgccctggagcccctggtggacctgcccatcggcatcaacatcaccagattccagaccctgctggccctgcacagaagctacctgacccccggcgacagcagcagcggctggaccgccggcgccgccgcctactacgtgggctacctgcagcccagaaccttcctgctgaagtacaacgagaacggcaccatcaccgacgccgtggactgcgccctggaccccctgagcgagaccaagtgcaccctgaagagcttcaccgtggagaagggcatctaccagaccagcaacttcagagtgcagcccaccgagagcatcgtgagattccccaacatcaccaacctgtgccccttcggcgaggtgttcaacgccaccagattcgccagcgtgtacgcctggaacagaaagagaatcagcaactgcgtggccgactacagcgtgctgtacaacagcgccagcttcagcaccttcaagtgctacggcgtgagccccaccaagctgaacgacctgtgcttcaccaacgtgtacgccgacagcttcgtgatcagaggcgacgaggtgagacagatcgcccccggccagaccggcaccatcgccgactacaactacaagctgcccgacgacttcaccggctgcgtgatcgcctggaacagcaacaacctggacagcaaggtgggcggcaactacaactacctgtacagactgttcagaaagagcaacctgaagcccttcgagagagacatcagcaccgagatctaccaggccggcagcaccccctgcaacggcgtgaagggcttcaactgctacttccccctgcagagctacggcttccagcccacctacggcgtgggctaccagccctacagagtggtggtgctgagcttcgagctgctgcacgcccccgccaccgtgtgcggccccaagaagagcaccaacctggtgaagaacaagtgcgtgaacttc

SEQ ID NO: 15 - DNA, 1623 bp, synthetic construct
  misc_feature 1..1623: note = For the preparation of mRNA vaccines
  source 1..1623: mol_type = other DNA
atgttcgtgttcctggtgctgctgcctctggtgagcagccagtgcgtgaacttcaccaacagaacccagctgcctagcgcctacaccaacagcttcaccagaggcgtgtactaccctgacaaggtgttcagaagcagcgtgctgcacagcacccaggacctgttcctgcctttcttcagcaacgtgacctggttccacgccatccacgtgagcggcaccaacggcaccaagagattcgacaaccctgtgctgcctttcaacgacggcgtgtacttcgccagcaccgagaagagcaacatcatcagaggctggatcttcggcaccaccctggacagcaagacccagagcctgctgatcgtgaacaacgccaccaacgtggtgatcaaggtgtgcgagttccagttctgcaactaccctttcctgggcgtgtactaccacaagaacaacaagagctggatggagagcgagttcagagtgtacagcagcgccaacaactgcaccttcgagtacgtgagccagcctttcctgatggacctggagggcaagcagggcaacttcaagaacctgagcgagttcgtgttcaagaacatcgacggctacttcaagatctacagcaagcacacccctatcaacctggtgagagacctgcctcagggcttcagcgccctggagcctctggtggacctgcctatcggcatcaacatcaccagattccagaccctgctggccctgcacagaagctacctgacccctggcgacagcagcagcggctggaccgccggcgccgccgcctactacgtgggctacctgcagcctagaaccttcctgctgaagtacaacgagaacggcaccatcaccgacgccgtggactgcgccctggaccctctgagcgagaccaagtgcaccctgaagagcttcaccgtggagaagggcatctaccagaccagcaacttcagagtgcagcctaccgagagcatcgtgagattccctaacatcaccaacctgtgccctttcggcgaggtgttcaacgccaccagattcgccagcgtgtacgcctggaacagaaagagaatcagcaactgcgtggccgactacagcgtgctgtacaacagcgccagcttcagcaccttcaagtgctacggcgtgagccctaccaagctgaacgacctgtgcttcaccaacgtgtacgccgacagcttcgtgatcagaggcgacgaggtgagacagatcgcccctggccagaccggcaccatcgccgactacaactacaagctgcctgacgacttcaccggctgcgtgatcgcctggaacagcaacaacctggacagcaaggtgggcggcaactacaactacctgtacagactgttcagaaagagcaacctgaagcctttcgagagagacatcagcaccgagatctaccaggccggcagcaccccttgcaacggcgtgaagggcttcaactgctacttccctctgcagagctacggcttccagcctacctacggcgtgggctaccagccttacagagtggtggtgctgagcttcgagctgctgcacgcccctgccaccgtgtgcggccctaagaagagcaccaacctggtgaagaacaagtgcgtgaacttc

SEQ ID NO: 16 - DNA, 1623 bp, synthetic construct
  misc_feature 1..1623: note = For the preparation of mRNA vaccines
  source 1..1623: mol_type = other DNA
atgttcgtgttcctggtgctgctgcccctggtgagcagccagtgcgtgaacttcaccaacaggacccagctgcccagcgcctacaccaacagcttcaccaggggcgtgtactaccccgacaaggtgttcaggagcagcgtgctgcacagcacccaggacctgttcctgcccttcttcagcaacgtgacctggttccacgccatccacgtgagcggcaccaacggcaccaagaggttcgacaaccccgtgctgcccttcaacgacggcgtgtacttcgccagcaccgagaagagcaacatcatcaggggctggatcttcggcaccaccctggacagcaagacccagagcctgctgatcgtgaacaacgccaccaacgtggtgatcaaggtgtgcgagttccagttctgcaactaccccttcctgggcgtgtactaccacaagaacaacaagagctggatggagagcgagttcagggtgtacagcagcgccaacaactgcaccttcgagtacgtgagccagcccttcctgatggacctggagggcaagcagggcaacttcaagaacctgagcgagttcgtgttcaagaacatcgacggctacttcaagatctacagcaagcacacccccatcaacctggtgagggacctgccccagggcttcagcgccctggagcccctggtggacctgcccatcggcatcaacatcaccaggttccagaccctgctggccctgcacaggagctacctgacccccggcgacagcagcagcggctggaccgccggcgccgccgcctactacgtgggctacctgcagcccaggaccttcctgctgaagtacaacgagaacggcaccatcaccgacgccgtggactgcgccctggaccccctgagcgagaccaagtgcaccctgaagagcttcaccgtggagaagggcatctaccagaccagcaacttcagggtgcagcccaccgagagcatcgtgaggttccccaacatcaccaacctgtgccccttcggcgaggtgttcaacgccaccaggttcgccagcgtgtacgcctggaacaggaagaggatcagcaactgcgtggccgactacagcgtgctgtacaacagcgccagcttcagcaccttcaagtgctacggcgtgagccccaccaagctgaacgacctgtgcttcaccaacgtgtacgccgacagcttcgtgatcaggggcgacgaggtgaggcagatcgcccccggccagaccggcaccatcgccgactacaactacaagctgcccgacgacttcaccggctgcgtgatcgcctggaacagcaacaacctggacagcaaggtgggcggcaactacaactacctgtacaggctgttcaggaagagcaacctgaagcccttcgagagggacatcagcaccgagatctaccaggccggcagcaccccctgcaacggcgtgaagggcttcaactgctacttccccctgcagagctacggcttccagcccacctacggcgtgggctaccagccctacagggtggtggtgctgagcttcgagctgctgcacgcccccgccaccgtgtgcggccccaagaagagcaccaacctggtgaagaacaagtgcgtgaacttc

SEQ ID NO: 17 - protein, 541 aa, synthetic construct
  REGION 1..541: note = Antigen
MFVFLVLLPLVSSQCVNLTTRTQLPPAYTNSFTRGVYYPDKVFRSSVLHSTQDLFLPFFSNVTWFHAIHVSGTNGTKRFDNPVLPFNDGVYFASTEKSNIIRGWIFGTTLDSKTQSLLIVNNATNVVIKVCEFQFCNDPFLGVYYHKNNKSWMESEFRVYSSANNCTFEYVSQPFLMDLEGKQGNFKNLREFVFKNIDGYFKIYSKHTPINLVRDLPQGFSALEPLVDLPIGINITRFQTLLALHRSYLTPGDSSSGWTAGAAAYYVGYLQPRTFLLKYNENGTITDAVDCALDPLSETKCTLKSFTVEKGIYQTSNFRVQPTESIVRFPNITNLCPFGEVFNATRFASVYAWNRKRISNCVADYSVLYNSASFSTFKCYGVSPTKLNDLCFTNVYADSFVIRGDEVRQIAPGQTGKIADYNYKLPDDFTGCVIAWNSNNLDSKVGGNYNYRYRLFRKSNLKPFERDISTEIYQAGSTPCNGVEGFNCYFPLQSYGFQPTNGVGYQPYRVVVLSFELLHAPATVCGPKKSTNLVKNKCVNF

SEQ ID NO: 18 - DNA, 1623 bp, synthetic construct
  misc_feature 1..1623: note = For the preparation of mRNA vaccines
  source 1..1623: mol_type = other DNA
atgttcgtgttcctggtgctgctgcccctggtgagcagccagtgcgtgaacctgaccaccagaacccagctgccccccgcctacaccaacagcttcaccagaggcgtgtactaccccgacaaggtgttcagaagcagcgtgctgcacagcacccaggacctgttcctgcccttcttcagcaacgtgacctggttccacgccatccacgtgagcggcaccaacggcaccaagagattcgacaaccccgtgctgcccttcaacgacggcgtgtacttcgccagcaccgagaagagcaacatcatcagaggctggatcttcggcaccaccctggacagcaagacccagagcctgctgatcgtgaacaacgccaccaacgtggtgatcaaggtgtgcgagttccagttctgcaacgaccccttcctgggcgtgtactaccacaagaacaacaagagctggatggagagcgagttcagagtgtacagcagcgccaacaactgcaccttcgagtacgtgagccagcccttcctgatggacctggagggcaagcagggcaacttcaagaacctgagagagttcgtgttcaagaacatcgacggctacttcaagatctacagcaagcacacccccatcaacctggtgagagacctgccccagggcttcagcgccctggagcccctggtggacctgcccatcggcatcaacatcaccagattccagaccctgctggccctgcacagaagctacctgacccccggcgacagcagcagcggctggaccgccggcgccgccgcctactacgtgggctacctgcagcccagaaccttcctgctgaagtacaacgagaacggcaccatcaccgacgccgtggactgcgccctggaccccctgagcgagaccaagtgcaccctgaagagcttcaccgtggagaagggcatctaccagaccagcaacttcagagtgcagcccaccgagagcatcgtgagattccccaacatcaccaacctgtgccccttcggcgaggtgttcaacgccaccagattcgccagcgtgtacgcctggaacagaaagagaatcagcaactgcgtggccgactacagcgtgctgtacaacagcgccagcttcagcaccttcaagtgctacggcgtgagccccaccaagctgaacgacctgtgcttcaccaacgtgtacgccgacagcttcgtgatcagaggcgacgaggtgagacagatcgcccccggccagaccggcaagatcgccgactacaactacaagctgcccgacgacttcaccggctgcgtgatcgcctggaacagcaacaacctggacagcaaggtgggcggcaactacaactacagatacagactgttcagaaagagcaacctgaagcccttcgagagagacatcagcaccgagatctaccaggccggcagcaccccctgcaacggcgtggagggcttcaactgctacttccccctgcagagctacggcttccagcccaccaacggcgtgggctaccagccctacagagtggtggtgctgagcttcgagctgctgcacgcccccgccaccgtgtgcggccccaagaagagcaccaacctggtgaagaacaagtgcgtgaacttc

SEQ ID NO: 19 - DNA, 1623 bp, synthetic construct
  misc_feature 1..1623: note = For the preparation of mRNA vaccines
  source 1..1623: mol_type = other DNA
atgttcgtgttcctggtgctgctgcctctggtgagcagccagtgcgtgaacctgaccaccagaacccagctgcctcctgcctacaccaacagcttcaccagaggcgtgtactaccctgacaaggtgttcagaagcagcgtgctgcacagcacccaggacctgttcctgcctttcttcagcaacgtgacctggttccacgccatccacgtgagcggcaccaacggcaccaagagattcgacaaccctgtgctgcctttcaacgacggcgtgtacttcgccagcaccgagaagagcaacatcatcagaggctggatcttcggcaccaccctggacagcaagacccagagcctgctgatcgtgaacaacgccaccaacgtggtgatcaaggtgtgcgagttccagttctgcaacgaccctttcctgggcgtgtactaccacaagaacaacaagagctggatggagagcgagttcagagtgtacagcagcgccaacaactgcaccttcgagtacgtgagccagcctttcctgatggacctggagggcaagcagggcaacttcaagaacctgagagagttcgtgttcaagaacatcgacggctacttcaagatctacagcaagcacacccctatcaacctggtgagagacctgcctcagggcttcagcgccctggagcctctggtggacctgcctatcggcatcaacatcaccagattccagaccctgctggccctgcacagaagctacctgacccctggcgacagcagcagcggctggaccgccggcgccgccgcctactacgtgggctacctgcagcctagaaccttcctgctgaagtacaacgagaacggcaccatcaccgacgccgtggactgcgccctggaccctctgagcgagaccaagtgcaccctgaagagcttcaccgtggagaagggcatctaccagaccagcaacttcagagtgcagcctaccgagagcatcgtgagattccctaacatcaccaacctgtgccctttcggcgaggtgttcaacgccaccagattcgccagcgtgtacgcctggaacagaaagagaatcagcaactgcgtggccgactacagcgtgctgtacaacagcgccagcttcagcaccttcaagtgctacggcgtgagccctaccaagctgaacgacctgtgcttcaccaacgtgtacgccgacagcttcgtgatcagaggcgacgaggtgagacagatcgcccctggccagaccggcaagatcgccgactacaactacaagctgcctgacgacttcaccggctgcgtgatcgcctggaacagcaacaacctggacagcaaggtgggcggcaactacaactacagatacagactgttcagaaagagcaacctgaagcctttcgagagagacatcagcaccgagatctaccaggccggcagcaccccttgcaacggcgtggagggcttcaactgctacttccctctgcagagctacggcttccagcctaccaacggcgtgggctaccagccttacagagtggtggtgctgagcttcgagctgctgcacgcccctgccaccgtgtgcggccctaagaagagcaccaacctggtgaagaacaagtgcgtgaacttc

SEQ ID NO: 20 - DNA, 1623 bp, synthetic construct
  misc_feature 1..1623: note = For the preparation of mRNA vaccines
  source 1..1623: mol_type = other DNA
atgttcgtgttcctggtgctgctgcccctggtgagcagccagtgcgtgaacctgaccaccaggacccagctgccccccgcctacaccaacagcttcaccaggggcgtgtactaccccgacaaggtgttcaggagcagcgtgctgcacagcacccaggacctgttcctgcccttcttcagcaacgtgacctggttccacgccatccacgtgagcggcaccaacggcaccaagaggttcgacaaccccgtgctgcccttcaacgacggcgtgtacttcgccagcaccgagaagagcaacatcatcaggggctggatcttcggcaccaccctggacagcaagacccagagcctgctgatcgtgaacaacgccaccaacgtggtgatcaaggtgtgcgagttccagttctgcaacgaccccttcctgggcgtgtactaccacaagaacaacaagagctggatggagagcgagttcagggtgtacagcagcgccaacaactgcaccttcgagtacgtgagccagcccttcctgatggacctggagggcaagcagggcaacttcaagaacctgagggagttcgtgttcaagaacatcgacggctacttcaagatctacagcaagcacacccccatcaacctggtgagggacctgccccagggcttcagcgccctggagcccctggtggacctgcccatcggcatcaacatcaccaggttccagaccctgctggccctgcacaggagctacctgacccccggcgacagcagcagcggctggaccgccggcgccgccgcctactacgtgggctacctgcagcccaggaccttcctgctgaagtacaacgagaacggcaccatcaccgacgccgtggactgcgccctggaccccctgagcgagaccaagtgcaccctgaagagcttcaccgtggagaagggcatctaccagaccagcaacttcagggtgcagcccaccgagagcatcgtgaggttccccaacatcaccaacctgtgccccttcggcgaggtgttcaacgccaccaggttcgccagcgtgtacgcctggaacaggaagaggatcagcaactgcgtggccgactacagcgtgctgtacaacagcgccagcttcagcaccttcaagtgctacggcgtgagccccaccaagctgaacgacctgtgcttcaccaacgtgtacgccgacagcttcgtgatcaggggcgacgaggtgaggcagatcgcccccggccagaccggcaagatcgccgactacaactacaagctgcccgacgacttcaccggctgcgtgatcgcctggaacagcaacaacctggacagcaaggtgggcggcaactacaactacaggtacaggctgttcaggaagagcaacctgaagcccttcgagagggacatcagcaccgagatctaccaggccggcagcaccccctgcaacggcgtggagggcttcaactgctacttccccctgcagagctacggcttccagcccaccaacggcgtgggctaccagccctacagggtggtggtgctgagcttcgagctgctgcacgcccccgccaccgtgtgcggccccaagaagagcaccaacctggtgaagaacaagtgcgtgaacttc

SEQ ID NO: 21 - protein, 538 aa, synthetic construct
  REGION 1..538: note = Antigen
MFVFLVLLPLVSSQCVNLTTRTQLPPAYTNSFTRGVYYPDKVFRSSVLHSTQDLFLPFFSNVTWFHVISGTNGTKRFDNPVLPFNDGVYFASIEKSNIIRGWIFGTTLDSKTQSLLIVNNATNVVIKVCEFQFCNDPFLDHKNNKSWMESEFRVYSSANNCTFEYVSQPFLMDLEGKQGNFKNLREFVFKNIDGYFKIYSKHTPIIVREPEDLPQGFSALEPLVDLPIGINITRFQTLLALHRSYLTPGDSSSGWTAGAAAYYVGYLQPRTFLLKYNENGTITDAVDCALDPLSETKCTLKSFTVEKGIYQTSNFRVQPTESIVRFPNITNLCPFDEVFNATRFASVYAWNRKRISNCVADYSVLYNLAPFFTFKCYGVSPTKLNDLCFTNVYADSFVIRGDEVRQIAPGQTGNIADYNYKLPDDFTGCVIAWNSNKLDSKVSGNYNYLYRLFRKSNLKPFERDISTEIYQAGNKPCNGVAGFNCYFPLRSYSFRPTYGVGHQPYRVVVLSFELLHAPATVCGPKKSTNLVKNKCVNF

SEQ ID NO: 22 - DNA, 1620 bp, synthetic construct
  misc_feature 1..1620: note = For the preparation of mRNA vaccines
  source 1..1620: mol_type = other DNA
atgtttgtgttcctggtgctgctgcccctggtgagcagccagtgcgtgaacctgaccaccagaacacagctgcctcccgcctacaccaactccttcacccgcggcgtgtactaccctgataaggtgttcaggagctccgtgctgcacagcacccaggacctgttcctgcctttcttctctaacgtgacctggttccacgtgattagcggcacaaacggcaccaagcggttcgataaccccgtgctgcccttcaacgacggcgtgtacttcgcctccatcgaaaaaagcaacattatcagaggctggatcttcggcaccaccctggattccaagacccagtccctgctgatcgtgaacaacgccaccaacgtcgtgatcaaggtgtgtgagttccagttctgtaatgaccccttcctggaccacaagaacaacaagagctggatggagagcgagttcagggtgtacagctccgccaacaactgcacattcgagtacgtgagccagcccttcctgatggacctggagggcaagcagggcaacttcaagaatctgagagagttcgtgttcaagaacatcgatggatacttcaagatctacagcaagcacacccctatcatcgtgagggagcctgaggacctgccccagggcttcagcgccctggagcccctcgtggacctgcctatcggcatcaacatcacaaggttccagaccctgctggccctgcacaggtcctacctgacaccaggcgacagcagcagcggctggacagccggcgccgccgcctactatgtgggctacctgcagcccagaacattcctgctgaagtataacgagaatggcaccatcacagacgccgtggactgtgccctggatcccctgagcgagaccaagtgcactctgaagtcctttacagtggagaagggaatctaccagacaagcaatttcagggtgcagcctacagagagcattgtgagattccctaacatcaccaacctgtgcccctttgacgaagtgtttaacgctacacggtttgcatcagtgtatgcctggaacaggaagagaatcagtaactgtgtggccgactactctgtgctgtataacctggctcccttctttactttcaaatgctacggggtgagccctactaagctgaatgacctgtgtttcacaaacgtgtatgccgatagctttgtgatcaggggcgacgaagtgagacagatcgctccaggccagacaggcaatattgccgattacaactataaactgcccgatgacttcacaggatgcgtgattgcctggaatagcaataagctggattctaaagtgagcggcaattacaattacctgtataggctgttcagaaagagcaacctgaagcctttcgagagagacatctccactgaaatctatcaggccggcaataagccctgcaacggcgtggctggctttaattgttactttcccctgagatcctatagctttcgccccacctatggcgtgggacaccagccttacagagtggtggtgctgtccttcgagctgctgcacgcccctgccacagtgtgcggcccaaagaagtccaccaatctggtgaagaataagtgcgtgaacttctgataa

SEQ ID NO: 23 - DNA, 1614 bp, synthetic construct
  misc_feature 1..1614: note = For the preparation of mRNA vaccines
  source 1..1614: mol_type = other DNA
atgttcgtgttcctggtgctgctgcctctggtgagcagccagtgcgtgaacctgaccaccaggacccagctgcctcctgcctacaccaacagcttcaccaggggcgtgtactaccctgacaaggtgttcaggagcagcgtgctgcacagcacccaggacctgttcctgcctttcttcagcaacgtgacctggttccacgtgatcagcggcaccaacggcaccaagaggttcgacaaccctgtgctgcctttcaacgacggcgtgtacttcgccagcatcgagaagagcaacatcatcaggggctggatcttcggcaccaccctggacagcaagacccagagcctgctgatcgtgaacaacgccaccaacgtggtgatcaaggtgtgcgagttccagttctgcaacgaccctttcctggaccacaagaacaacaagagctggatggagagcgagttcagggtgtacagcagcgccaacaactgcaccttcgagtacgtgagccagcctttcctgatggacctggagggcaagcagggcaacttcaagaacctgagggagttcgtgttcaagaacatcgacggctacttcaagatctacagcaagcacacccctatcctggtgagggagcctgaggacctgcctcagggcttcagcgccctggagcctctggtggacctgcctatcggcatcaacatcaccaggttccagaccctgctggccctgcacaggagctacctgacccctggcgacagcagcagcggctggaccgccggcgccgccgcctactacgtgggctacctgcagcctaggaccttcctgctgaagtacaacgagaacggcaccatcaccgacgccgtggactgcgccctggaccctctgagcgagaccaagtgcaccctgaagagcttcaccgtggagaagggcatctaccagaccagcaacttcagggtgcagcctaccgagagcatcgtgaggttccctaacatcaccaacctgtgccctttcgacgaggtgttcaacgccaccaggttcgccagcgtgtacgcctggaacaggaagaggatcagcaactgcgtggccgactacagcgtgctgtacaacctggcccctttcttcaccttcaagtgctacggcgtgagccctaccaagctgaacgacctgtgcttcaccaacgtgtacgccgacagcttcgtgatcaggggcgacgaggtgaggcagatcgcccctggccagaccggcaacatcgccgactacaactacaagctgcctgacgacttcaccggctgcgtgatcgcctggaacagcaacaagctggacagcaaggtgagcggcaactacaactacctgtacaggctgttcaggaagagcaacctgaagcctttcgagagggacatcagcaccgagatctaccaggccggcaacaagccttgcaacggcgtggccggcttcaactgctacttccctctgaggagctacagcttcaggcctacctacggcgtgggccaccagccttacagggtggtggtgctgagcttcgagctgctgcacgcccctgccaccgtgtgcggccctaagaagagcaccaacctggtgaagaacaagtgcgtgaacttc

SEQ ID NO: 24 - DNA, 1614 bp, synthetic construct
  misc_feature 1..1614: note = For the preparation of mRNA vaccines
  source 1..1614: mol_type = other DNA
atgttcgtgttcctggtgctgctgcccctggtgagcagccagtgcgtgaacctgaccaccaggacccagctgccccccgcctacaccaacagcttcaccaggggcgtgtactaccccgacaaggtgttcaggagcagcgtgctgcacagcacccaggacctgttcctgcccttcttcagcaacgtgacctggttccacgtgatcagcggcaccaacggcaccaagaggttcgacaaccccgtgctgcccttcaacgacggcgtgtacttcgccagcatcgagaagagcaacatcatcaggggctggatcttcggcaccaccctggacagcaagacccagagcctgctgatcgtgaacaacgccaccaacgtggtgatcaaggtgtgcgagttccagttctgcaacgaccccttcctggaccacaagaacaacaagagctggatggagagcgagttcagggtgtacagcagcgccaacaactgcaccttcgagtacgtgagccagcccttcctgatggacctggagggcaagcagggcaacttcaagaacctgagggagttcgtgttcaagaacatcgacggctacttcaagatctacagcaagcacacccccatcctggtgagggagcccgaggacctgccccagggcttcagcgccctggagcccctggtggacctgcccatcggcatcaacatcaccaggttccagaccctgctggccctgcacaggagctacctgacccccggcgacagcagcagcggctggaccgccggcgccgccgcctactacgtgggctacctgcagcccaggaccttcctgctgaagtacaacgagaacggcaccatcaccgacgccgtggactgcgccctggaccccctgagcgagaccaagtgcaccctgaagagcttcaccgtggagaagggcatctaccagaccagcaacttcagggtgcagcccaccgagagcatcgtgaggttccccaacatcaccaacctgtgccccttcgacgaggtgttcaacgccaccaggttcgccagcgtgtacgcctggaacaggaagaggatcagcaactgcgtggccgactacagcgtgctgtacaacctggcccccttcttcaccttcaagtgctacggcgtgagccccaccaagctgaacgacctgtgcttcaccaacgtgtacgccgacagcttcgtgatcaggggcgacgaggtgaggcagatcgcccccggccagaccggcaacatcgccgactacaactacaagctgcccgacgacttcaccggctgcgtgatcgcctggaacagcaacaagctggacagcaaggtgagcggcaactacaactacctgtacaggctgttcaggaagagcaacctgaagcccttcgagagggacatcagcaccgagatctaccaggccggcaacaagccctgcaacggcgtggccggcttcaactgctacttccccctgaggagctacagcttcaggcccacctacggcgtgggccaccagccctacagggtggtggtgctgagcttcgagctgctgcacgcccccgccaccgtgtgcggccccaagaagagcaccaacctggtgaagaacaagtgcgtgaacttc

SEQ ID NO: 25 - RNA, 1623 nt, synthetic construct
  misc_feature 1..1623: note = mRNAvaccines
  source 1..1623: mol_type = other RNA
atgttcgtgttcctggtgctgctgcccctggtgagcagccagtgcgtgaacctgaccaccaggacccagctgccccccgcctacaccaacagcttcaccaggggcgtgtactaccccgacaaggtgttcaggagcagcgtgctgcacagcacccaggacctgttcctgcccttcttcagcaacgtgacctggttccacgccatccacgtgagcggcaccaacggcaccaagaggttcgacaaccccgtgctgcccttcaacgacggcgtgtacttcgccagcaccgagaagagcaacatcatcaggggctggatcttcggcaccaccctggacagcaagacccagagcctgctgatcgtgaacaacgccaccaacgtggtgatcaaggtgtgcgagttccagttctgcaacgaccccttcctgggcgtgtactaccacaagaacaacaagagctggatggagagcgagttcagggtgtacagcagcgccaacaactgcaccttcgagtacgtgagccagcccttcctgatggacctggagggcaagcagggcaacttcaagaacctgagggagttcgtgttcaagaacatcgacggctacttcaagatctacagcaagcacacccccatcaacctggtgagggacctgccccagggcttcagcgccctggagcccctggtggacctgcccatcggcatcaacatcaccaggttccagaccctgctggccctgcacaggagctacctgacccccggcgacagcagcagcggctggaccgccggcgccgccgcctactacgtgggctacctgcagcccaggaccttcctgctgaagtacaacgagaacggcaccatcaccgacgccgtggactgcgccctggaccccctgagcgagaccaagtgcaccctgaagagcttcaccgtggagaagggcatctaccagaccagcaacttcagggtgcagcccaccgagagcatcgtgaggttccccaacatcaccaacctgtgccccttcggcgaggtgttcaacgccaccaggttcgccagcgtgtacgcctggaacaggaagaggatcagcaactgcgtggccgactacagcgtgctgtacaacagcgccagcttcagcaccttcaagtgctacggcgtgagccccaccaagctgaacgacctgtgcttcaccaacgtgtacgccgacagcttcgtgatcaggggcgacgaggtgaggcagatcgcccccggccagaccggcaagatcgccgactacaactacaagctgcccgacgacttcaccggctgcgtgatcgcctggaacagcaacaacctggacagcaaggtgggcggcaactacaactacctgtacaggctgttcaggaagagcaacctgaagcccttcgagagggacatcagcaccgagatctaccaggccggcagcaccccctgcaacggcgtggagggcttcaactgctacttccccctgcagagctacggcttccagcccaccaacggcgtgggctaccagccctacagggtggtggtgctgagcttcgagctgctgcacgcccccgccaccgtgtgcggccccaagaagagcaccaacctggtgaagaacaagtgcgtgaacttc

SEQ ID NO: 26 - RNA, 1623 nt, synthetic construct
  misc_feature 1..1623: note = mRNAvaccines
  source 1..1623: mol_type = other RNA
atgttcgtgttcctggtgctgctgcctctggtgagcagccagtgcgtgaacctgaccaccagaacccagctgcctcctgcctacaccaacagcttcaccagaggcgtgtactaccctgacaaggtgttcagaagcagcgtgctgcacagcacccaggacctgttcctgcctttcttcagcaacgtgacctggttccacgccatccacgtgagcggcaccaacggcaccaagagattcgacaaccctgtgctgcctttcaacgacggcgtgtacttcgccagcaccgagaagagcaacatcatcagaggctggatcttcggcaccaccctggacagcaagacccagagcctgctgatcgtgaacaacgccaccaacgtggtgatcaaggtgtgcgagttccagttctgcaacgaccctttcctgggcgtgtactaccacaagaacaacaagagctggatggagagcgagttcagagtgtacagcagcgccaacaactgcaccttcgagtacgtgagccagcctttcctgatggacctggagggcaagcagggcaacttcaagaacctgagagagttcgtgttcaagaacatcgacggctacttcaagatctacagcaagcacacccctatcaacctggtgagagacctgcctcagggcttcagcgccctggagcctctggtggacctgcctatcggcatcaacatcaccagattccagaccctgctggccctgcacagaagctacctgacccctggcgacagcagcagcggctggaccgccggcgccgccgcctactacgtgggctacctgcagcctagaaccttcctgctgaagtacaacgagaacggcaccatcaccgacgccgtggactgcgccctggaccctctgagcgagaccaagtgcaccctgaagagcttcaccgtggagaagggcatctaccagaccagcaacttcagagtgcagcctaccgagagcatcgtgagattccctaacatcaccaacctgtgccctttcggcgaggtgttcaacgccaccagattcgccagcgtgtacgcctggaacagaaagagaatcagcaactgcgtggccgactacagcgtgctgtacaacagcgccagcttcagcaccttcaagtgctacggcgtgagccctaccaagctgaacgacctgtgcttcaccaacgtgtacgccgacagcttcgtgatcagaggcgacgaggtgagacagatcgcccctggccagaccggcaagatcgccgactacaactacaagctgcctgacgacttcaccggctgcgtgatcgcctggaacagcaacaacctggacagcaaggtgggcggcaactacaactacctgtacagactgttcagaaagagcaacctgaagcctttcgagagagacatcagcaccgagatctaccaggccggcagcaccccttgcaacggcgtggagggcttcaactgctacttccctctgcagagctacggcttccagcctaccaacggcgtgggctaccagccttacagagtggtggtgctgagcttcgagctgctgcacgcccctgccaccgtgtgcggccctaagaagagcaccaacctggtgaagaacaagtgcgtgaacttc

SEQ ID NO: 27 - RNA, 1623 nt, synthetic construct; identical to SEQ ID NO: 25
  misc_feature 1..1623: note = mRNAvaccines
  source 1..1623: mol_type = other RNA

SEQ ID NO: 28 - RNA, 1614 nt, synthetic construct
  misc_feature 1..1614: note = mRNAvaccines
  source 1..1614: mol_type = other RNA
atgttcgtgttcctggtgctgctgcccctggtgagcagccagtgcgtgaacctgaccaccagaacccagctgccccccgcctacaccaacagcttcaccagaggcgtgtactaccccgacaaggtgttcagaagcagcgtgctgcacagcacccaggacctgttcctgcccttcttcagcaacgtgacctggttccacgccatcagcggcaccaacggcaccaagagattcgacaaccccgtgctgcccttcaacgacggcgtgtacttcgccagcaccgagaagagcaacatcatcagaggctggatcttcggcaccaccctggacagcaagacccagagcctgctgatcgtgaacaacgccaccaacgtggtgatcaaggtgtgcgagttccagttctgcaacgaccccttcctgggcgtgtaccacaagaacaacaagagctggatggagagcgagttcagagtgtacagcagcgccaacaactgcaccttcgagtacgtgagccagcccttcctgatggacctggagggcaagcagggcaacttcaagaacctgagagagttcgtgttcaagaacatcgacggctacttcaagatctacagcaagcacacccccatcaacctggtgagagacctgccccagggcttcagcgccctggagcccctggtggacctgcccatcggcatcaacatcaccagattccagaccctgctggccctgcacagaagctacctgacccccggcgacagcagcagcggctggaccgccggcgccgccgcctactacgtgggctacctgcagcccagaaccttcctgctgaagtacaacgagaacggcaccatcaccgacgccgtggactgcgccctggaccccctgagcgagaccaagtgcaccctgaagagcttcaccgtggagaagggcatctaccagaccagcaacttcagagtgcagcccaccgagagcatcgtgagattccccaacatcaccaacctgtgccccttcggcgaggtgttcaacgccaccagattcgccagcgtgtacgcctggaacagaaagagaatcagcaactgcgtggccgactacagcgtgctgtacaacagcgccagcttcagcaccttcaagtgctacggcgtgagccccaccaagctgaacgacctgtgcttcaccaacgtgtacgccgacagcttcgtgatcagaggcgacgaggtgagacagatcgcccccggccagaccggcaagatcgccgactacaactacaagctgcccgacgacttcaccggctgcgtgatcgcctggaacagcaacaacctggacagcaaggtgggcggcaactacaactacctgtacagactgttcagaaagagcaacctgaagcccttcgagagagacatcagcaccgagatctaccaggccggcagcaccccctgcaacggcgtggagggcttcaactgctacttccccctgcagagctacggcttccagcccacctacggcgtgggctaccagccctacagagtggtggtgctgagcttcgagctgctgcacgcccccgccaccgtgtgcggccccaagaagagcaccaacctggtgaagaacaagtgcgtgaacttc

SEQ ID NO: 29 - RNA, 1614 nt, synthetic construct
  misc_feature 1..1614: note = mRNAvaccines
  source 1..1614: mol_type = other RNA
atgttcgtgttcctggtgctgctgcctctggtgagcagccagtgcgtgaacctgaccaccagaacccagctgcctcctgcctacaccaacagcttcaccagaggcgtgtactaccctgacaaggtgttcagaagcagcgtgctgcacagcacccaggacctgttcctgcctttcttcagcaacgtgacctggttccacgccatcagcggcaccaacggcaccaagagattcgacaaccctgtgctgcctttcaacgacggcgtgtacttcgccagcaccgagaagagcaacatcatcagaggctggatcttcggcaccaccctggacagcaagacccagagcctgctgatcgtgaacaacgccaccaacgtggtgatcaaggtgtgcgagttccagttctgcaacgaccctttcctgggcgtgtaccacaagaacaacaagagctggatggagagcgagttcagagtgtacagcagcgccaacaactgcaccttcgagtacgtgagccagcctttcctgatggacctggagggcaagcagggcaacttcaagaacctgagagagttcgtgttcaagaacatcgacggctacttcaagatctacagcaagcacacccctatcaacctggtgagagacctgcctcagggcttcagcgccctggagcctctggtggacctgcctatcggcatcaacatcaccagattccagaccctgctggccctgcacagaagctacctgacccctggcgacagcagcagcggctggaccgccggcgccgccgcctactacgtgggctacctgcagcctagaaccttcctgctgaagtacaacgagaacggcaccatcaccgacgccgtggactgcgccctggaccctctgagcgagaccaagtgcaccctgaagagcttcaccgtggagaagggcatctaccagaccagcaacttcagagtgcagcctaccgagagcatcgtgagattccctaacatcaccaacctgtgccctttcggcgaggtgttcaacgccaccagattcgccagcgtgtacgcctggaacagaaagagaatcagcaactgcgtggccgactacagcgtgctgtacaacagcgccagcttcagcaccttcaagtgctacggcgtgagccctaccaagctgaacgacctgtgcttcaccaacgtgtacgccgacagcttcgtgatcagaggcgacgaggtgagacagatcgcccctggccagaccggcaagatcgccgactacaactacaagctgcctgacgacttcaccggctgcgtgatcgcctggaacagcaacaacctggacagcaaggtgggcggcaactacaactacctgtacagactgttcagaaagagcaacctgaagcctttcgagagagacatcagcaccgagatctaccaggccggcagcaccccttgcaacggcgtggagggcttcaactgctacttccctctgcagagctacggcttccagcctacctacggcgtgggctaccagccttacagagtggtggtgctgagcttcgagctgctgcacgcccctgccaccgtgtgcggccctaagaagagcaccaacctggtgaagaacaagtgcgtgaacttc

SEQ ID NO: 30 - RNA, 1614 nt, synthetic construct
  misc_feature 1..1614: note = mRNAvaccines
  source 1..1614: mol_type = other RNA
atgttcgtgttcctggtgctgctgcccctggtgagcagccagtgcgtgaacctgaccaccaggacccagctgccccccgcctacaccaacagcttcaccaggggcgtgtactaccccgacaaggtgttcaggagcagcgtgctgcacagcacccaggacctgttcctgcccttcttcagcaacgtgacctggttccacgccatcagcggcaccaacggcaccaagaggttcgacaaccccgtgctgcccttcaacgacggcgtgtacttcgccagcaccgagaagagcaacatcatcaggggctggatcttcggcaccaccctggacagcaagacccagagcctgctgatcgtgaacaacgccaccaacgtggtgatcaaggtgtgcgagttccagttctgcaacgaccccttcctgggcgtgtaccacaagaacaacaagagctggatggagagcgagttcagggtgtacagcagcgccaacaactgcaccttcgagtacgtgagccagcccttcctgatggacctggagggcaagcagggcaacttcaagaacctgagggagttcgtgttcaagaacatcgacggctacttcaagatctacagcaagcacacccccatcaacctggtgagggacctgccccagggcttcagcgccctggagcccctggtggacctgcccatcggcatcaacatcaccaggttccagaccctgctggccctgcacaggagctacctgacccccggcgacagcagcagcggctggaccgccggcgccgccgcctactacgtgggctacctgcagcccaggaccttcctgctgaagtacaacgagaacggcaccatcaccgacgccgtggactgcgccctggaccccctgagcgagaccaagtgcaccctgaagagcttcaccgtggagaagggcatctaccagaccagcaacttcagggtgcagcccaccgagagcatcgtgaggttccccaacatcaccaacctgtgccccttcggcgaggtgttcaacgccaccaggttcgccagcgtgtacgcctggaacaggaagaggatcagcaactgcgtggccgactacagcgtgctgtacaacagcgccagcttcagcaccttcaagtgctacggcgtgagccccaccaagctgaacgacctgtgcttcaccaacgtgtacgccgacagcttcgtgatcaggggcgacgaggtgaggcagatcgcccccggccagaccggcaagatcgccgactacaactacaagctgcccgacgacttcaccggctgcgtgatcgcctggaacagcaacaacctggacagcaaggtgggcggcaactacaactacctgtacaggctgttcaggaagagcaacctgaagcccttcgagagggacatcagcaccgagatctaccaggccggcagcaccccctgcaacggcgtggagggcttcaactgctacttccccctgcagagctacggcttccagcccacctacggcgtgggctaccagccctacagggtggtggtgctgagcttcgagctgctgcacgcccccgccaccgtgtgcggccccaagaagagcaccaacctggtgaagaacaagtgcgtgaacttc

SEQ ID NO: 31 - RNA, 1617 nt, synthetic construct
  misc_feature 1..1617: note = mRNAvaccines
  source 1..1617: mol_type = other RNA
atgttcgtgttcctggtgctgctgcccctggtgagcagccagtgcgtgaacctgaccaccaggacccagctgccccccgcctacaccaacagcttcaccaggggcgtgtactaccccgacaaggtgttcaggagcagcgtgctgcacagcacccaggacctgttcctgcccttcttcagcaacgtgacctggttccacgccatccacgtgagcggcaccaacggcaccaagaggttcgccaaccccgtgctgcccttcaacgacggcgtgtacttcgccagcaccgagaagagcaacatcatcaggggctggatcttcggcaccaccctggacagcaagacccagagcctgctgatcgtgaacaacgccaccaacgtggtgatcaaggtgtgcgagttccagttctgcaacgaccccttcctgggcgtgtactaccacaagaacaacaagagctggatggagagcgagttcagggtgtacagcagcgccaacaactgcaccttcgagtacgtgagccagcccttcctgatggacctggagggcaagcagggcaacttcaagaacctgagggagttcgtgttcaagaacatcgacggctacttcaagatctacagcaagcacacccccatcaacctggtgaggggcctgccccagggcttcagcgccctggagcccctggtggacctgcccatcggcatcaacatcaccaggttccagaccctgctgcacaggagctacctgacccccggcgacagcagcagcggctggaccgccggcgccgccgcctactacgtgggctacctgcagcccaggaccttcctgctgaagtacaacgagaacggcaccatcaccgacgccgtggactgcgccctggaccccctgagcgagaccaagtgcaccctgaagagcttcaccgtggagaagggcatctaccagaccagcaacttcagggtgcagcccaccgagagcatcgtgaggttccccaacatcaccaacctgtgccccttcggcgaggtgttcaacgccaccaggttcgccagcgtgtacgcctggaacaggaagaggatcagcaactgcgtggccgactacagcgtgctgtacaacagcgccagcttcagcaccttcaagtgctacggcgtgagccccaccaagctgaacgacctgtgcttcaccaacgtgtacgccgacagcttcgtgatcaggggcgacgaggtgaggcagatcgcccccggccagaccggcaacatcgccgactacaactacaagctgcccgacgacttcaccggctgcgtgatcgcctggaacagcaacaacctggacagcaaggtgggcggcaactacaactacctgtacaggctgttcaggaagagcaacctgaagcccttcgagagggacatcagcaccgagatctaccaggccggcagcaccccctgcaacggcgtgaagggcttcaactgctacttccccctgcagagctacggcttccagcccacctacggcgtgggctaccagccctacagggtggtggtgctgagcttcgagctgctgcacgcccccgccaccgtgtgcggccccaagaagagcaccaacctggtgaagaacaagtgcgtgaacttc

SEQ ID NO: 32 - RNA, 1617 nt, synthetic construct
  misc_feature 1..1617: note = mRNAvaccines
  source 1..1617: mol_type = other RNA
atgttcgtgttcctggtgctgctgcctctggtgagcagccagtgcgtgaacctgaccaccaggacccagctgcctcctgcctacaccaacagcttcaccaggggcgtgtactaccctgacaaggtgttcaggagcagcgtgctgcacagcacccaggacctgttcctgcctttcttcagcaacgtgacctggttccacgccatccacgtgagcggcaccaacggcaccaagaggttcgccaaccctgtgctgcctttcaacgacggcgtgtacttcgccagcaccgagaagagcaacatcatcaggggctggatcttcggcaccaccctggacagcaagacccagagcctgctgatcgtgaacaacgccaccaacgtggtgatcaaggtgtgcgagttccagttctgcaacgaccctttcctgggcgtgtactaccacaagaacaacaagagctggatggagagcgagttcagggtgtacagcagcgccaacaactgcaccttcgagtacgtgagccagcctttcctgatggacctggagggcaagcagggcaacttcaagaacctgagggagttcgtgttcaagaacatcgacggctacttcaagatctacagcaagcacacccctatcaacctggtgaggggcctgcctcagggcttcagcgccctggagcctctggtggacctgcctatcggcatcaacatcaccaggttccagaccctgctgcacaggagctacctgacccctggcgacagcagcagcggctggaccgccggcgccgccgcctactacgtgggctacctgcagcctaggaccttcctgctgaagtacaacgagaacggcaccatcaccgacgccgtggactgcgccctggaccctctgagcgagaccaagtgcaccctgaagagcttcaccgtggagaagggcatctaccagaccagcaacttcagggtgcagcctaccgagagcatcgtgaggttccctaacatcaccaacctgtgccctttcggcgaggtgttcaacgccaccaggttcgccagcgtgtacgcctggaacaggaagaggatcagcaactgcgtggccgactacagcgtgctgtacaacagcgccagcttcagcaccttcaagtgctacggcgtgagccctaccaagctgaacgacctgtgcttcaccaacgtgtacgccgacagcttcgtgatcaggggcgacgaggtgaggcagatcgcccctggccagaccggcaacatcgccgactacaactacaagctgcctgacgacttcaccggctgcgtgatcgcctggaacagcaacaacctggacagcaaggtgggcggcaactacaactacctgtacaggctgttcaggaagagcaacctgaagcctttcgagagggacatcagcaccgagatctaccaggccggcagcaccccttgcaacggcgtgaagggcttcaactgctacttccctctgcagagctacggcttccagcctacctacggcgtgggctaccagccttacagggtggtggtgctgagcttcgagctgctgcacgcccctgccaccgtgtgcggccctaagaagagcaccaacctggtgaagaacaagtgcgtgaacttc

SEQ ID NO: 33 - RNA, 1617 nt, synthetic construct; identical to SEQ ID NO: 31
  misc_feature 1..1617: note = mRNAvaccines
  source 1..1617: mol_type = other RNA

SEQ ID NO: 34 - RNA, 1623 nt, synthetic construct
  misc_feature 1..1623: note = mRNAvaccines
  source 1..1623: mol_type = other RNA
atgttcgtgttcctggtgctgctgcccctggtgagcagccagtgcgtgaacttcaccaacagaacccagctgcccagcgcctacaccaacagcttcaccagaggcgtgtactaccccgacaaggtgttcagaagcagcgtgctgcacagcacccaggacctgttcctgcccttcttcagcaacgtgacctggttccacgccatccacgtgagcggcaccaacggcaccaagagattcgacaaccccgtgctgcccttcaacgacggcgtgtacttcgccagcaccgagaagagcaacatcatcagaggctggatcttcggcaccaccctggacagcaagacccagagcctgctgatcgtgaacaacgccaccaacgtggtgatcaaggtgtgcgagttccagttctgcaactaccccttcctgggcgtgtactaccacaagaacaacaagagctggatggagagcgagttcagagtgtacagcagcgccaacaactgcaccttcgagtacgtgagccagcccttcctgatggacctggagggcaagcagggcaacttcaagaacctgagcgagttcgtgttcaagaacatcgacggctacttcaagatctacagcaagcacacccccatcaacctggtgagagacctgccccagggcttcagcgccctggagcccctggtggacctgcccatcggcatcaacatcaccagattccagaccctgctggccctgcacagaagctacctgacccccggcgacagcagcagcggctggaccgccggcgccgccgcctactacgtgggctacctgcagcccagaaccttcctgctgaagtacaacgagaacggcaccatcaccgacgccgtggactgcgccctggaccccctgagcgagaccaagtgcaccctgaagagcttcaccgtggagaagggcatctaccagaccagcaacttcagagtgcagcccaccgagagcatcgtgagattccccaacatcaccaacctgtgccccttcggcgaggtgttcaacgccaccagattcgccagcgtgtacgcctggaacagaaagagaatcagcaactgcgtggccgactacagcgtgctgtacaacagcgccagcttcagcaccttcaagtgctacggcgtgagccccaccaagctgaacgacctgtgcttcaccaacgtgtacgccgacagcttcgtgatcagaggcgacgaggtgagacagatcgcccccggccagaccggcaccatcgccgactacaactacaagctgcccgacgacttcaccggctgcgtgatcgcctggaacagcaacaacctggacagcaaggtgggcggcaactacaactacctgtacagactgttcagaaagagcaacctgaagcccttcgagagagacatcagcaccgagatctaccaggccggcagcaccccctgcaacggcgtgaagggcttcaactgctacttccccctgcagagctacggcttccagcccacctacggcgtgggctaccagccctacagagtggtggtgctgagcttcgagctgctgcacgcccccgccaccgtgtgcggccccaagaagagcaccaacctggtgaagaacaagtgcgtgaacttc

SEQ ID NO: 35 - RNA, 1623 nt, synthetic construct
  misc_feature 1..1623: note = mRNAvaccines
  source 1..1623: mol_type = other RNA
atgttcgtgttcctggtgctgctgcctctggtgagcagccagtgcgtgaacttcaccaacagaacccagctgcctagcgcctacaccaacagcttcaccagaggcgtgtactaccctgacaaggtgttcagaagcagcgtgctgcacagcacccaggacctgttcctgcctttcttcagcaacgtgacctggttccacgccatccacgtgagcggcaccaacggcaccaagagattcgacaaccctgtgctgcctttcaacgacggcgtgtacttcgccagcaccgagaagagcaacatcatcagaggctggatcttcggcaccaccctggacagcaagacccagagcctgctgatcgtgaacaacgccaccaacgtggtgatcaaggtgtgcgagttccagttctgcaactaccctttcctgggcgtgtactaccacaagaacaacaagagctggatggagagcgagttcagagtgtacagcagcgccaacaactgcaccttcgagtacgtgagccagcctttcctgatggacctggagggcaagcagggcaacttcaagaacctgagcgagttcgtgttcaagaacatcgacggctacttcaagatctacagcaagcacacccctatcaacctggtgagagacctgcctcagggcttcagcgccctggagcctctggtggacctgcctatcggcatcaacatcaccagattccagaccctgctggccctgcacagaagctacctgacccctggcgacagcagcagcggctggaccgccggcgccgccgcctactacgtgggctacctgcagcctagaaccttcctgctgaagtacaacgagaacggcaccatcaccgacgccgtggactgcgccctggaccctctgagcgagaccaagtgcaccctgaagagcttcaccgtggagaagggcatctaccagaccagcaacttcagagtgcagcctaccgagagcatcgtgagattccctaacatcaccaacctgtgccctttcggcgaggtgttcaacgccaccagattcgccagcgtgtacgcctggaacagaaagagaatcagcaactgcgtggccgactacagcgtgctgtacaacagcgccagcttcagcaccttcaagtgctacggcgtgagccctaccaagctgaacgacctgtgcttcaccaacgtgtacgccgacagcttcgtgatcagaggcgacgaggtgagacagatcgcccctggccagaccggcaccatcgccgactacaactacaagctgcctgacgacttcaccggctgcgtgatcgcctggaacagcaacaacctggacagcaaggtgggcggcaactacaactacctgtacagactgttcagaaagagcaacctgaagcctttcgagagagacatcagcaccgagatctaccaggccggcagcaccccttgcaacggcgtgaagggcttcaactgctacttccctctgcagagctacggcttccagcctacctacggcgtgggctaccagccttacagagtggtggtgctgagcttcgagctgctgcacgcccctgccaccgtgtgcggccctaagaagagcaccaacctggtgaagaacaagtgcgtgaacttc

SEQ ID NO: 36 - RNA, 1623 nt, synthetic construct
  misc_feature 1..1623: note = mRNAvaccines
  source 1..1623: mol_type = other RNA
atgttcgtgttcctggtgctgctgcccctggtgagcagccagtgcgtgaacttcaccaacaggacccagctgcccagcgcctacaccaacagcttcaccaggggcgtgtactaccccgacaaggtgttcaggagcagcgtgctgcacagcacccaggacctgttcctgcccttcttcagcaacgtgacctggttccacgccatccacgtgagcggcaccaacggcaccaagaggttcgacaaccccgtgctgcccttcaacgacggcgtgtacttcgccagcaccgagaagagcaacatcatcaggggctggatcttcggcaccaccctggacagcaagacccagagcctgctgatcgtgaacaacgccaccaacgtggtgatcaaggtgtgcgagttccagttctgcaactaccccttcctgggcgtgtactaccacaagaacaacaagagctggatggagagcgagttcagggtgtacagcagcgccaacaactgcaccttcgagtacgtgagccagcccttcctgatggacctggagggcaagcagggcaacttcaagaacctgagcgagttcgtgttcaagaacatcgacggctacttcaagatctacagcaagcacacccccatcaacctggtgagggacctgccccagggcttcagcgccctggagcccctggtggacctgcccatcggcatcaacatcaccaggttccagaccctgctggccctgcacaggagctacctgacccccggcgacagcagcagcggctggaccgccggcgccgccgcctactacgtgggctacctgcagcccaggaccttcctgctgaagtacaacgagaacggcaccatcaccgacgccgtggactgcgccctggaccccctgagcgagaccaagtgcaccctgaagagcttcaccgtggagaagggcatctaccagaccagcaacttcagggtgcagcccaccgagagcatcgtgaggttccccaacatcaccaacctgtgccccttcggcgaggtgttcaacgccaccaggttcgccagcgtgtacgcctggaacaggaagaggatcagcaactgcgtggccgactacagcgtgctgtacaacagcgccagcttcagcaccttcaagtgctacggcgtgagccccaccaagctgaacgacctgtgcttcaccaacgtgtacgccgacagcttcgtgatcaggggcgacgaggtgaggcagatcgcccccggccagaccggcaccatcgccgactacaactacaagctgcccgacgacttcaccggctgcgtgatcgcctggaacagcaacaacctggacagcaaggtgggcggcaactacaactacctgtacaggctgttcaggaagagcaacctgaagcccttcgagagggacatcagcaccgagatctaccaggccggcagcaccccctgcaacggcgtgaagggcttcaactgctacttccccctgcagagctacggcttccagcccacctacggcgtgggctaccagccctacagggtggtggtgctgagcttcgagctgctgcacgcccccgccaccgtgtgcggccccaagaagagcaccaacctggtgaagaacaagtgcgtgaacttc

SEQ ID NO: 37 - RNA, 1623 nt, synthetic construct
  misc_feature 1..1623: note = mRNAvaccines
  source 1..1623: mol_type = other RNA
atgttcgtgttcctggtgctgctgcccctggtgagcagccagtgcgtgaacctgaccaccagaacccagctgccccccgcctacaccaacagcttcaccagaggcgtgtactaccccgacaaggtgttcagaagcagcgtgctgcacagcacccaggacctgttcctgcccttcttcagcaacgtgacctggttccacgccatccacgtgagcggcaccaacggcaccaagagattcgacaaccccgtgctgcccttcaacgacggcgtgtacttcgccagcaccgagaagagcaacatcatcagaggctggatcttcggcaccaccctggacagcaagacccagagcctgctgatcgtgaacaacgccaccaacgtggtgatcaaggtgtgcgagttccagttctgcaacgaccccttcctgggcgtgtactaccacaagaacaacaagagctggatggagagcgagttcagagtgtacagcagcgccaacaactgcaccttcgagtacgtgagccagcccttcctgatggacctggagggcaagcagggcaacttcaagaacctgagagagttcgtgttcaagaacatcgacggctacttcaagatctacagcaagcacacccccatcaacctggtgagagacctgccccagggcttcagcgccctggagcccctggtggacctgcccatcggcatcaacatcaccagattccagaccctgctggccctgcacagaagctacctgacccccggcgacagcagcagcggctggaccgccggcgccgccgcctactacgtgggctacctgcagcccagaaccttcctgctgaagtacaacgagaacggcaccatcaccgacgccgtggactgcgccctggaccccctgagcgagaccaagtgcaccctgaagagcttcaccgtggagaagggcatctaccagaccagcaacttcagagtgcagcccaccgagagcatcgtgagattccccaacatcaccaacctgtgccccttcggcgaggtgttcaacgccaccagattcgccagcgtgtacgcctggaacagaaagagaatcagcaactgcgtggccgactacagcgtgctgtacaacagcgccagcttcagcaccttcaagtgctacggcgtgagccccaccaagctgaacgacctgtgcttcaccaacgtgtacgccgacagcttcgtgatcagaggcgacgaggtgagacagatcgcccccggccagaccggcaagatcgccgactacaactacaagctgcccgacgacttcaccggctgcgtgatcgcctggaacagcaacaacctggacagcaaggtgggcggcaactacaactacagatacagactgttcagaaagagcaacctgaagcccttcgagagagacatcagcaccgagatctaccaggccggcagcaccccctgcaacggcgtggagggcttcaactgctacttccccctgcagagctacggcttccagcccaccaacggcgtgggctaccagccctacagagtggtggtgctgagcttcgagctgctgcacgcccccgccaccgtgtgcggccccaagaagagcaccaacctggtgaagaacaagtgcgtgaacttc

SEQ ID NO: 38 - RNA, 1623 nt, synthetic construct
  misc_feature 1..1623: note = mRNAvaccines
  source 1..1623: mol_type = other RNA
atgttcgtgttcctggtgctgctgcctctggtgagcagccagtgcgtgaacctgaccaccagaacccagctgcctcctgcctacaccaacagcttcaccagaggcgtgtactaccctgacaaggtgttcagaagcagcgtgctgcacagcacccaggacctgttcctgcctttcttcagcaacgtgacctggttccacgccatccacgtgagcggcaccaacggcaccaagagattcgacaaccctgtgctgcctttcaacgacggcgtgtacttcgccagcaccgagaagagcaacatcatcagaggctggatcttcggcaccaccctggacagcaagacccagagcctgctgatcgtgaacaacgccaccaacgtggtgatcaaggtgtgcgagttccagttctgcaacgaccctttcctgggcgtgtactaccacaagaacaacaagagctggatggagagcgagttcagagtgtacagcagcgccaacaactgcaccttcgagtacgtgagccagcctttcctgatggacctggagggcaagcagggcaacttcaagaacctgagagagttcgtgttcaagaacatcgacggctacttcaagatctacagcaagcacacccctatcaacctggtgagagacctgcctcagggcttcagcgccctggagcctctggtggacctgcctatcggcatcaacatcaccagattccagaccctgctggccctgcacagaagctacctgacccctggcgacagcagcagcggctggaccgccggcgccgccgcctactacgtgggctacctgcagcctagaaccttcctgctgaagtacaacgagaacggcaccatcaccgacgccgtggactgcgccctggaccctctgagcgagaccaagtgcaccctgaagagcttcaccgtggagaagggcatctaccagaccagcaacttcagagtgcagcctaccgagagcatcgtgagattccctaacatcaccaacctgtgccctttcggcgaggtgttcaacgccaccagattcgccagcgtgtacgcctggaacagaaagagaatcagcaactgcgtggccgactacagcgtgctgtacaacagcgccagcttcagcaccttcaagtgctacggcgtgagccctaccaagctgaacgacctgtgcttcaccaacgtgtacgccgacagcttcgtgatcagaggcgacgaggtgagacagatcgcccctggccagaccggcaagatcgccgactacaactacaagctgcctgacgacttcaccggctgcgtgatcgcctggaacagcaacaacctggacagcaaggtgggcggcaactacaactacagatacagactgttcagaaagagcaacctgaagcctttcgagagagacatcagcaccgagatctaccaggccggcagcaccccttgcaacggcgtggagggcttcaactgctacttccctctgcagagctacggcttccagcctaccaacggcgtgggctaccagccttacagagtggtggtgctgagcttcgagctgctgcacgcccctgccaccgtgtgcggccctaagaagagcaccaacctggtgaagaacaagtgcgtgaacttc

SEQ ID NO: 39 - RNA, 1623 nt, synthetic construct
  misc_feature 1..1623: note = mRNAvaccines
  source 1..1623: mol_type = other RNA
atgttcgtgttcctggtgctgctgcccctggtgagcagccagtgcgtgaacctgaccaccaggacccagctgccccccgcctacaccaacagcttcaccaggggcgtgtactaccccgacaaggtgttcaggagcagcgtgctgcacagcacccaggacctgttcctgcccttcttcagcaacgtgacctggttccacgccatccacgtgagcggcaccaacggcaccaagaggttcgacaaccccgtgctgcccttcaacgacggcgtgtacttcgccagcaccgagaagagcaacatcatcaggggctggatcttcggcaccaccctggacagcaagacccagagcctgctgatcgtgaacaacgccaccaacgtggtgatcaaggtgtgcgagttccagttctgcaacgaccccttcctgggcgtgtactaccacaagaacaacaagagctggatggagagcgagttcagggtgtacagcagcgccaacaactgcaccttcgagtacgtgagccagcccttcctgatggacctggagggcaagcagggcaacttcaagaacctgagggagttcgtgttcaagaacatcgacggctacttcaagatctacagcaagcacacccccatcaacctggtgagggacctgccccagggcttcagcgccctggagcccctggtggacctgcccatcggcatcaacatcaccaggttccagaccctgctggccctgcacaggagctacctgacccccggcgacagcagcagcggctggaccgccggcgccgccgcctactacgtgggctacctgcagcccaggaccttcctgctgaagtacaacgagaacggcaccatcaccgacgccgtggactgcgccctggaccccctgagcgagaccaagtgcaccctgaagagcttcaccgtggagaagggcatctaccagaccagcaacttcagggtgcagcccaccgagagcatcgtgaggttccccaacatcaccaacctgtgccccttcggcgaggtgttcaacgccaccaggttcgccagcgtgtacgcctggaacaggaagaggatcagcaactgcgtggccgactacagcgtgctgtacaacagcgccagcttcagcaccttcaagtgctacggcgtgagccccaccaagctgaacgacctgtgcttcaccaacgtgtacgccgacagcttcgtgatcaggggcgacgaggtgaggcagatcgcccccggccagaccggcaagatcgccgactacaactacaagctgcccgacgacttcaccggctgcgtgatcgcctggaacagcaacaacctggacagcaaggtgggcggcaactacaactacaggtacaggctgttcaggaagagcaacctgaagcccttcgagagggacatcagcaccgagatctaccaggccggcagcaccccctgcaacggcgtggagggcttcaactgctacttccccctgcagagctacggcttccagcccaccaacggcgtgggctaccagccctacagggtggtggtgctgagcttcgagctgctgcacgcccccgccaccgtgtgcggccccaagaagagcaccaacctggtgaagaacaagtgcgtgaacttc

SEQ ID NO: 40 - RNA, 1620 nt, synthetic construct
  misc_feature 1..1620: note = mRNAvaccines
  source 1..1620: mol_type = other RNA
atgtttgtgttcctggtgctgctgcccctggtgagcagccagtgcgtgaacctgaccaccagaacacagctgcctcccgcctacaccaactccttcacccgcggcgtgtactaccctgataaggtgttcaggagctccgtgctgcacagcacccaggacctgttcctgcctttcttctctaacgtgacctggttccacgtgattagcggcacaaacggcaccaagcggttcgataaccccgtgctgcccttcaacgacggcgtgtacttcgcctccatcgaaaaaagcaacattatcagaggctggatcttcggcaccaccctggattccaagacccagtccctgctgatcgtgaacaacgccaccaacgtcgtgatcaaggtgtgtgagttccagttctgtaatgaccccttcctggaccacaagaacaacaagagctggatggagagcgagttcagggtgtacagctccgccaacaactgcacattcgagtacgtgagccagcccttcctgatggacctggagggcaagcagggcaacttcaagaatctgagagagttcgtgttcaagaacatcgatggatacttcaagatctacagcaagcacacccctatcatcgtgagggagcctgaggacctgccccagggcttcagcgccctggagcccctcgtggacctgcctatcggcatcaacatcacaaggttccagaccctgctggccctgcacaggtcctacctgacaccaggcgacagcagcagcggctggacagccggcgccgccgcctactatgtgggctacctgcagcccagaacattcctgctgaagtataacgagaatggcaccatcacagacgccgtggactgtgccctggatcccctgagcgagaccaagtgcactctgaagtcctttacagtggagaagggaatctaccagacaagcaatttcagggtgcagcctacagagagcattgtgagattccctaacatcaccaacctgtgcccctttgacgaagtgtttaacgctacacggtttgcatcagtgtatgcctggaacaggaagagaatcagtaactgtgtggccgactactctgtgctgtataacctggctcccttctttactttcaaatgctacggggtgagccctactaagctgaatgacctgtgtttcacaaacgtgtatgccgatagctttgtgatcaggggcgacgaagtgagacagatcgctccaggccagacaggcaatattgccgattacaactataaactgcccgatgacttcacaggatgcgtgattgcctggaatagcaataagctggattctaaagtgagcggcaattacaattacctgtataggctgttcagaaagagcaacctgaagcctttcgagagagacatctccactgaaatctatcaggccggcaataagccctgcaacggcgtggctggctttaattgttactttcccctgagatcctatagctttcgccccacctatggcgtgggacaccagccttacagagtggtggtgctgtccttcgagctgctgcacgcccctgccacagtgtgcggcccaaagaagtccaccaatctggtgaagaataagtgcgtgaacttctgataa

SEQ ID NO: 41 - RNA, 1614 nt, synthetic construct
  misc_feature 1..1614: note = mRNAvaccines
  source 1..1614: mol_type = other RNA
atgttcgtgttcctggtgctgctgcccctggtgagcagccagtgcgtgaacctgaccaccaggacccagctgccccccgcctacaccaacagcttcaccaggggcgtgtactaccccgacaaggtgttcaggagcagcgtgctgcacagcacccaggacctgttcctgcccttcttcagcaacgtgacctggttccacgtgatcagcggcaccaacggcaccaagaggttcgacaaccccgtgctgcccttcaacgacggcgtgtacttcgccagcatcgagaagagcaacatcatcaggggctggatcttcggcaccaccctggacagcaagacccagagcctgctgatcgtgaacaacgccaccaacgtggtgatcaaggtgtgcgagttccagttctgcaacgaccccttcctggaccacaagaacaacaagagctggatggagagcgagttcagggtgtacagcagcgccaacaactgcaccttcgagtacgtgagccagcccttcctgatggacctggagggcaagcagggcaacttcaagaacctgagggagttcgtgttcaagaacatcgacggctacttcaagatctacagcaagcacacccccatcctggtgagggagcccgaggacctgccccagggcttcagcgccctggagcccctggtggacctgcccatcggcatcaacatcaccaggttccagaccctgctggccctgcacaggagctacctgacccccggcgacagcagcagcggctggaccgccggcgccgccgcctactacgtgggctacctgcagcccaggaccttcctgctgaagtacaacgagaacggcaccatcaccgacgccgtggactgcgccctggaccccctgagcgagaccaagtgcaccctgaagagcttcaccgtggagaagggcatctaccagaccagcaacttcagggtgcagcccaccgagagcatcgtgaggttccccaacatcaccaacctgtgccccttcgacgaggtgttcaacgccaccaggttcgccagcgtgtacgcctggaacaggaagaggatcagcaactgcgtggccgactacagcgtgctgtacaacctggcccccttcttcaccttcaagtgctacggcgtgagccccaccaagctgaacgacctgtgcttcaccaacgtgtacgccgacagcttcgtgatcaggggcgacgaggtgaggcagatcgcccccggccagaccggcaacatcgccgactacaactacaagctgcccgacgacttcaccggctgcgtgatcgcctggaacagcaacaagctggacagcaaggtgagcggcaactacaactacctgtacaggctgttcaggaagagcaacctgaagcccttcgagagggacatcagcaccgagatctaccaggccggcaacaagccctgcaacggcgtggccggcttcaactgctacttccccctgaggagctacagcttcaggcccacctacggcgtgggccaccagccctacagggtggtggtgctgagcttcgagctgctgcacgcccccgccaccgtgtgcggccccaagaagagcaccaacctggtgaagaacaagtgcgtgaacttc

SEQ ID NO: 42 - RNA, 1614 nt, synthetic construct; identical to SEQ ID NO: 41
  misc_feature 1..1614: note = mRNAvaccines
  source 1..1614: mol_type = other RNA

SEQ ID NO: 43 - RNA, 672 nt, synthetic construct
  misc_feature 1..672: note = mRNAvaccines
  source 1..672: mol_type = other RNA
atgagggtgcagcccaccgagagcatcgtgaggttccccaacatcaccaacctgtgccccttcggcgaggtgttcaacgccaccaggttcgccagcgtgtacgcctggaacaggaagaggatcagcaactgcgtggccgactacagcgtgctgtacaacagcgccagcttcagcaccttcaagtgctacggcgtgagccccaccaagctgaacgacctgtgcttcaccaacgtgtacgccgacagcttcgtgatcaggggcgacgaggtgaggcagatcgcccccggccagaccggcaagatcgccgactacaactacaagctgcccgacgacttcaccggctgcgtgatcgcctggaacagcaacaacctggacagcaaggtgggcggcaactacaactacctgtacaggctgttcaggaagagcaacctgaagcccttcgagagggacatcagcaccgagatctaccaggccggcagcaccccctgcaacggcgtggagggcttcaactgctacttccccctgcagagctacggcttccagcccaccaacggcgtgggctaccagccctacagggtggtggtgctgagcttcgagctgctgcacgcccccgccaccgtgtgcggccccaagaagagcaccaacctggtgaagaacaagtgcgtgaacttc

SEQ ID NO: 44 - protein, 529 aa, synthetic construct
  REGION 1..529: note = NTD-RBD
SQCVNLTTRTQLPPAYTNSFTRGVYYPDKVFRSSVLHSTQDLFLPFFSNVTWFHAIHVSGTNGTKRFDNPVLPFNDGVYFASTEKSNIIRGWIFGTTLDSKTQSLLIVNNATNVVIKVCEFQFCNDPFLGVYYHKNNKSWMESEFRVYSSANNCTFEYVSQPFLMDLEGKQGNFKNLREFVFKNIDGYFKIYSKHTPINLVRDLPQGFSALEPLVDLPIGINITRFQTLLALHRSYLTPGDSSSGWTAGAAAYYVGYLQPRTFLLKYNENGTITDAVDCALDPLSETKCTLKSFTVEKGIYQTSNFRVQPTESIVRFPNITNLCPFGEVFNATRFASVYAWNRKRISNCVADYSVLYNSASFSTFKCYGVSPTKLNDLCFTNVYADSFVIRGDEVRQIAPGQTGKIADYNYKLPDDFTGCVIAWNSNNLDSKVGGNYNYLYRLFRKSNLKPFERDISTEIYQAGSTPCNGVEGFNCYFPLQSYGFQPTNGVGYQPYRVVVLSFELLHAPATVCGPKKSTNLVKNKCVNF

SEQ ID NO: 45 - protein, 526 aa, synthetic construct
  REGION 1..526: note = NTD-RBD
SQCVNLTTRTQLPPAYTNSFTRGVYYPDKVFRSSVLHSTQDLFLPFFSNVTWFHAISGTNGTKRFDNPVLPFNDGVYFASTEKSNIIRGWIFGTTLDSKTQSLLIVNNATNVVIKVCEFQFCNDPFLGVYHKNNKSWMESEFRVYSSANNCTFEYVSQPFLMDLEGKQGNFKNLREFVFKNIDGYFKIYSKHTPINLVRDLPQGFSALEPLVDLPIGINITRFQTLLALHRSYLTPGDSSSGWTAGAAAYYVGYLQPRTFLLKYNENGTITDAVDCALDPLSETKCTLKSFTVEKGIYQTSNFRVQPTESIVRFPNITNLCPFGEVFNATRFASVYAWNRKRISNCVADYSVLYNSASFSTFKCYGVSPTKLNDLCFTNVYADSFVIRGDEVRQIAPGQTGKIADYNYKLPDDFTGCVIAWNSNNLDSKVGGNYNYLYRLFRKSNLKPFERDISTEIYQAGSTPCNGVEGFNCYFPLQSYGFQPTYGVGYQPYRVVVLSFELLHAPATVCGPKKSTNLVKNKCVNF

SEQ ID NO: 46 - protein, 527 aa, synthetic construct
  REGION 1..527: note = NTD-RBD
SQCVNLTTRTQLPPAYTNSFTRGVYYPDKVFRSSVLHSTQDLFLPFFSNVTWFHAIHVSGTNGTKRFANPVLPFNDGVYFASTEKSNIIRGWIFGTTLDSKTQSLLIVNNATNVVIKVCEFQFCNDPFLGVYYHKNNKSWMESEFRVYSSANNCTFEYVSQPFLMDLEGKQGNFKNLREFVFKNIDGYFKIYSKHTPINLVRGLPQGFSALEPLVDLPIGINITRFQTLLHRSYLTPGDSSSGWTAGAAAYYVGYLQPRTFLLKYNENGTITDAVDCALDPLSETKCTLKSFTVEKGIYQTSNFRVQPTESIVRFPNITNLCPFGEVFNATRFASVYAWNRKRISNCVADYSVLYNSASFSTFKCYGVSPTKLNDLCFTNVYADSFVIRGDEVRQIAPGQTGNIADYNYKLPDDFTGCVIAWNSNNLDSKVGGNYNYLYRLFRKSNLKPFERDISTEIYQAGSTPCNGVKGFNCYFPLQSYGFQPTYGVGYQPYRVVVLSFELLHAPATVCGPKKSTNLVKNKCVNF

SEQ ID NO: 47 - protein, 529 aa, synthetic construct
  REGION 1..529: note = NTD-RBD
SQCVNFTNRTQLPSAYTNSFTRGVYYPDKVFRSSVLHSTQDLFLPFFSNVTWFHAIHVSGTNGTKRFDNPVLPFNDGVYFASTEKSNIIRGWIFGTTLDSKTQSLLIVNNATNVVIKVCEFQFCNYPFLGVYYHKNNKSWMESEFRVYSSANNCTFEYVSQPFLMDLEGKQGNFKNLSEFVFKNIDGYFKIYSKHTPINLVRDLPQGFSALEPLVDLPIGINITRFQTLLALHRSYLTPGDSSSGWTAGAAAYYVGYLQPRTFLLKYNENGTITDAVDCALDPLSETKCTLKSFTVEKGIYQTSNFRVQPTESIVRFPNITNLCPFGEVFNATRFASVYAWNRKRISNCVADYSVLYNSASFSTFKCYGVSPTKLNDLCFTNVYADSFVIRGDEVRQIAPGQTGTIADYNYKLPDDFTGCVIAWNSNNLDSKVGGNYNYLYRLFRKSNLKPFERDISTEIYQAGSTPCNGVKGFNCYFPLQSYGFQPTYGVGYQPYRVVVLSFELLHAPATVCGPKKSTNLVKNKCVNF

SEQ ID NO: 48 - protein, 529 aa, synthetic construct
  REGION 1..529: note = NTD-RBD
SQCVNLTTRTQLPPAYTNSFTRGVYYPDKVFRSSVLHSTQDLFLPFFSNVTWFHAIHVSGTNGTKRFDNPVLPFNDGVYFASTEKSNIIRGWIFGTTLDSKTQSLLIVNNATNVVIKVCEFQFCNDPFLGVYYHKNNKSWMESEFRVYSSANNCTFEYVSQPFLMDLEGKQGNFKNLREFVFKNIDGYFKIYSKHTPINLVRDLPQGFSALEPLVDLPIGINITRFQTLLALHRSYLTPGDSSSGWTAGAAAYYVGYLQPRTFLLKYNENGTITDAVDCALDPLSETKCTLKSFTVEKGIYQTSNFRVQPTESIVRFPNITNLCPFGEVFNATRFASVYAWNRKRISNCVADYSVLYNSASFSTFKCYGVSPTKLNDLCFTNVYADSFVIRGDEVRQIAPGQTGKIADYNYKLPDDFTGCVIAWNSNNLDSKVGGNYNYRYRLFRKSNLKPFERDISTEIYQAGSTPCNGVEGFNCYFPLQSYGFQPTNGVGYQPYRVVVLSFELLHAPATVCGPKKSTNLVKNKCVNF

SEQ ID NO: 49 - protein, 526 aa, synthetic construct
  REGION 1..526: note = NTD-RBD
SQCVNLTTRTQLPPAYTNSFTRGVYYPDKVFRSSVLHSTQDLFLPFFSNVTWFHVISGTNGTKRFDNPVLPFNDGVYFASIEKSNIIRGWIFGTTLDSKTQSLLIVNNATNVVIKVCEFQFCNDPFLDHKNNKSWMESEFRVYSSANNCTFEYVSQPFLMDLEGKQGNFKNLREFVFKNIDGYFKIYSKHTPIIVREPEDLPQGFSALEPLVDLPIGINITRFQTLLALHRSYLTPGDSSSGWTAGAAAYYVGYLQPRTFLLKYNENGTITDAVDCALDPLSETKCTLKSFTVEKGIYQTSNFRVQPTESIVRFPNITNLCPFDEVFNATRFASVYAWNRKRISNCVADYSVLYNLAPFFTFKCYGVSPTKLNDLCFTNVYADSFVIRGDEVRQIAPGQTGNIADYNYKLPDDFTGCVIAWNSNKLDSKVSGNYNYLYRLFRKSNLKPFERDISTEIYQAGNKPCNGVAGFNCYFPLRSYSFRPTYGVGHQPYRVVVLSFELLHAPATVCGPKKSTNLVKNKCVNF

SEQ ID NO: 50 - protein, 14 aa, synthetic construct
  REGION 1..14: note = linking peptide
SFTVEKGIYQTSNF

SEQ ID NO: 51 - RNA, 51 nt, synthetic construct
  misc_feature 1..51: note = 5'UTR
  source 1..51: mol_type = other RNA
agggagataagagagaaaagaagagtaagaagaaatataagagccgccacc

SEQ ID NO: 52 - RNA, 93 nt, synthetic construct
  misc_feature 1..93: note = 3'UTR
  source 1..93: mol_type = other RNA
gctgccttctgcggggcttgccttctggccatgcccttcttctctcccttgcacctgtacctcttggtctttgaataaagcctgagtaggaag

SEQ ID NO: 53 - RNA, 112 nt, synthetic construct
  misc_feature 1..112: note = Poly-A tail
  source 1..112: mol_type = other RNA
aaaaaaaaaaaaaaaaaaaaaaaaaaaaaaagcatatgactaaaaaaaaaaaaaaaaaaaaaaaaaaaaaaaaaaaaaaaaaaaaaaaaaaaaaaaaaaaaaaaaaaaaaaa

SEQ ID NO: 54 - RNA, 1614 nt, synthetic construct
  misc_feature 1..1614: note = mRNAvaccines
  source 1..1614: mol_type = other RNA
atgttcgtgttcctggtgctgctgccgttagtgagtagtcagtgtgtgaacctgactactcgcacgcagctgccaccagcgtacacgaacagcttcacgcggggcgtgtattatcccgacaaagtatttcgcagcagcgtcctgcactccacccaggacctcttcctcccgttcttctccaatgtgacgtggtttcacgtcatatcggggacgaacgggacgaagaggttcgacaatccggtcctgccttttaacgacggggtgtatttcgcgtcaatagagaagagtaatattatccgagggtggatcttcgggaccaccctggatagtaagactcagtctctattgatcgtgaataacgccaccaacgtcgttataaaggtctgcgagtttcagttctgcaatgatccattcttggatcataagaacaataagtcgtggatggagagcgagtttcgagtgtactcgagtgcaaacaattgcactttcgagtacgtctcgcagccgttcttgatggacctggagggtaagcaggggaatttcaagaatcttagagaattcgtctttaagaatattgacggatactttaagatttattccaagcatacccctattatcgtccgggagccggaggacctgccgcagggcttcagcgctctggagccgctggttgacctcccgatagggatcaacatcacgcggttccagacgctgttagccctgcacaggtcctacctgactcccggcgatagtagttctgggtggactgcaggcgctgctgcgtactatgtcgggtacttacagccccgcacgttcttgttgaagtacaacgagaacggcacaatcacggacgccgttgattgtgccctagatccgttatcggagaccaagtgtactctcaagtcgttcaccgtggagaagggcatctaccagacgtccaacttcagggtgcagccgactgagagtatagttcggtttccgaacataacgaatctatgcccgtttgacgaggtgttcaatgcgacgcgcttcgcctccgtgtatgcatggaaccgaaaacgcataagcaattgtgtcgcagattattcagttttgtacaatctcgccccgttcttcacgttcaagtgttacggggtgagtccgacaaagctgaatgatctgtgtttcacaaatgtttatgcggattcgttcgtgatacgcggagacgaagtgcgtcagattgctcctggtcagacgggcaatatagccgactataactacaagctaccagacgacttcactggttgtgtgatagcttggaattcgaacaagctggacagcaaggtatcaggtaattacaattacctgtaccggctgttcaggaagtcgaatttgaagcctttcgagcgcgacatctcgaccgagatctaccaggccggaaacaagccgtgcaacggagtagcaggcttcaactgctactttccgttgcgcagctacagtttccggcctacctacggggtagggcaccagccctaccgcgtagtggtgctctccttcgagctgctccacgcaccggccacggtgtgtgggccgaagaagagcaccaatctggtcaagaacaagtgcgtgaacttt

SEQ ID NO: 55 - RNA, 1614 nt, synthetic construct
  misc_feature 1..1614: note = mRNAvaccines
  source 1..1614: mol_type = other RNA
atgttcgtcttcctggtgctgcttccgctggtcagttcacagtgtgtgaacttgaccacgcggacgcagctaccccccgcgtatacgaactcgtttacgcggggggtatattacccggataaggtgtttcgtagttccgttctccacagtactcaggacctcttcctcccgttcttctccaatgtgacgtggtttcacgtcatatcggggacgaacgggacgaagaggttcgacaaccccgtgttgcccttcaacgacggggtttatttcgcgtcaatagagaagagtaatattatccgagggtggatcttcgggaccaccctggatagtaagactcagtctctattgatcgtgaacaacgccactaatgtggtgatcaaggtgtgcgagtttcagttctgcaatgatccattcttggatcataagaacaacaagagttggatggagagtgaattccgtgtttactcttcagccaacaattgtaccttcgagtatgtcagtcagccgtttctgatggatcttgaaggcaagcagggcaatttcaagaatttgcgcgagtttgtcttcaagaacatcgacggctacttcaagatatactcgaagcacacgccgataattgtgcgcgagccggaagatctaccacagggcttcagtgctctggagcccttggtagatcttccgatcggcataaatatcacgcgtttccagacgctgctggcgttgcaccggagttaccttactccgggcgactccagcagcggctggacggcaggggctgcagcgtactatgtagggtatctgcaaccgcgcacgttcttgttgaagtacaacgagaacggcacgattacagatgccgtagattgtgcgctggaccccctgtcggagactaagtgcaccttgaagagttttactgtggagaagggaatctaccagacatctaacttccgggtgcagccgacagagagtattgtacgtttcccgaacatcacgaatctatgcccgtttgacgaggtgtttaacgccacgcggtttgctagtgtgtatgcgtggaatcgcaagcgcattagcaactgcgtggcggattattcagttttgtataatctcgccccgttcttcacgttcaagtgttacggggtgagtcctacaaagctgaatgatctctgcttcaccaacgtctacgcggatagctttgttatccgcggagacgaggtgaggcagatagcacctggtcagacgggcaatattgctgactacaactataagctcccggatgacttcaccgggtgcgttatagcgtggaacagcaataagttagattcgaaggtgtcgggaaactacaattatctctatcggctgttcaggaagtcgaacttaaagccttttgagcgtgatatatctaccgagatatatcaggctgggaataagccgtgcaacggggtagcaggcttcaactgctacttcccgttgcgcagctattcctttcggcccacctacggggtagggcaccagccctaccgcgtagttgtactgtcgtttgagctgctgcatgctccagcgacagtatgtgggccgaagaagtcgacgaacttggtgaagaacaagtgcgtcaacttc